European Patent Specification EP 3 585 417 B1, published February 22, 2023. Title: NOVEL CODON-OPTIMIZED CFTR MRNA. Applicant: Translate Bio Inc. The sequence listing filed with the application follows.

SEQUENCE LISTING (40 sequences)

SEQ ID NO: 1 - RNA, 4443 nt, Synthetic Oligonucleotide
augcaacgcucuccucuugaaaaggccucggugguguccaagcucuucuucucguggacuagacccauccugagaaagggguacagacagcgcuuggagcuguccgauaucuaucaaaucccuuccguggacuccgcggacaaccuguccgagaagcucgagagagaaugggacagagaacucgccucaaagaagaacccgaagcugauuaaugcgcuuaggcggugcuuuuucuggcgguucauguucuacggcaucuuccucuaccugggagaggucaccaaggccgugcagccccuguugcugggacggauuauugccuccuacgaccccgacaacaaggaagaaagaagcaucgcuaucuacuugggcaucggucugugccugcuuuucaucguccggacccucuuguugcauccugcuauuuucggccugcaucacauuggcaugcagaugagaauugccauguuuucccugaucuacaagaaaacucugaagcucucgagccgcgugcuugacaagauuuccaucggccagcucgugucccugcucuccaacaaucugaacaaguucgacgagggccucgcccuggcccacuucguguggaucgccccucugcaaguggcgcuucugaugggccugaucugggagcugcugcaagccucggcauucugugggcuuggauuccugaucgugcuggcacuguuccaggccggacuggggcggaugaugaugaaguacagggaccagagagccggaaagauuuccgaacggcuggugaucacuucggaaaugaucgaaaacauccagucagugaaggccuacugcugggaagaggccauggaaaagaugauugaaaaccuccggcaaaccgagcugaagcugacccgcaaggccgcuuacgugcgcuauuucaacucguccgcuuucuucuucuccggguucuucgugguguuucucuccgugcuccccuacgcccugauuaagggaaucauccucaggaagaucuucaccaccauuuccuucuguaucgugcuccgcauggccgugacccggcaguucccaugggccgugcagacuugguacgacucccugggagccauuaacaagauccaggacuuccuucaaaagcaggaguacaagacccucgaguacaaccugacuacuaccgaggucgugauggaaaacgucaccgccuuuugggaggagggauuuggcgaacuguucgagaaggccaagcagaacaacaacaaccgcaagaccucgaacggugacgacucccucuucuuuucaaacuucagccugcucgggacgcccgugcugaaggacauuaacuucaagaucgaaagaggacagcuccuggcgguggccggaucgaccggagccggaaagacuucccugcugauggugaucaugggagagcuugaaccuagcgagggaaagaucaagcacuccggccgcaucagcuucuguagccaguuuuccuggaucaugcccggaaccauuaaggaaaacaucaucuucggcguguccuacgaugaauaccgcuaccgguccgugaucaaagccugccagcuggaagaggauauuucaaaguucgcggagaaagauaacaucgugcugggcgaaggggguauuaccuugucggggggccagcgggcuagaaucucgcuggccagagccguguauaaggacgccgaccuguaucuccuggacucccccuucggauaccuggacguccugaccgaaaaggagaucuucgaaucgugcgugugcaagcugauggcuaacaagacucgcauccucgugaccuccaaaauggagcaccugaagaaggcagacaagauucugauucugcaugagggguccuccuacuuuuacggcaccuucucggaguugcagaacuugcagcccgacuucucaucgaagcugauggguugcgacagcuucgaccaguucuccgccgaaagaaggaacucgauccugacggaaaccuugcaccgcuucucuuuggaaggcgacgccccugugucauggaccgagacuaagaagcagagcuucaagcagaccggggaauucggcgaaaagaggaagaacagcaucuugaaccccauuaacuccauccgcaaguucucaaucgugcaaaagacgccacugcagaugaacggcauugaggaggacuccgacgaaccccuugagaggcgccugucccuggugccggacagcgagcagggagaagccauccugccucggauuuccgugaucuccacugguccgacgcuccaagcccggcggcggcaguccgugcugaaccugaugacccacagcgugaaccagggccaaaacauucaccgcaagacuaccgcauccacccggaaagugucccuggcaccucaagcgaaucuuaccgagcucgacaucuacucccggagacugucgcaggaaaccgggcucgaaauuuccgaagaaaucaacgaggaggaucugaaagagugcuucuucgacgauauggagucgauacccgccgugacgacuuggaacacuuaucugcgguacaucacugugcacaagucauugaucuucgugcugauuuggugccuggugauuuuccuggccgaggucgcggccucacugguggugcucuggcuguugggaaacacgccucugcaagacaagggaaacuccacgcacucgagaaacaacagcuaugccgugauuaucacuuccaccuccucuuauuacguguucuacaucuacgucggaguggcggauacccugcucgcgauggguuucuucagaggacugccgcugguccacaccuugaucaccgucagcaagauucuucaccacaagauguugcauagcgugcugcaggcccccauguccacccucaacacucugaaggccggaggcauucugaacagauucuccaaggacaucgcuauccuggacgaucuccugccgcuuaccaucuuugacuucauccagcugcugcugaucgugauuggagcaaucgcagugguggcggugcugcagccuuacauuuucguggccacugugccggucauuguggcguucaucaugcugcgggccuacuuccuccaaaccagccagcagcugaagcaacuggaauccgagggacgaucccccaucuucacucaccuugugacgucguugaagggacuguggacccuccgggcuuucggacggcagcccuacuucgaaacccucuuccacaaggcccugaaccuccacaccgccaauugguuccuguaccuguccacccugcggugguuccagaugcgcaucgagaugauuuucgucaucuucuucaucgcggucacauucaucagcauccugacuaccggagagggagagggacgggucggaauaauccugacccucgccaugaacauuaugagcacccugcagugggcagugaacagcucgaucgacguggacagccugaugcgaagcgucagccgcguguucaaguucaucgacaugccuacugagggaaaacccacuaaguccacuaagcccuacaaaaauggccagcugagcaaggucaugaucaucgaaaacucccacgugaagaaggacgauauuuggcccuccggaggucaaaugaccgugaaggaccugaccgcaaaguacaccgagggaggaaacgccauucucgaaaacaucagcuucuccauuucgccgggacagcgggucggccuucucgggcggaccgguuccgggaagucaacucugcugucggcuuuccuccggcugcugaauaccgagggggaaauccaaauugacggcgugucuugggauuccauuacucugcagcaguggcggaaggccuucggcgugaucccccagaagguguucaucuucucggguaccuuccggaagaaccuggauccuuacgagcaguggagcgaccaagaaaucuggaaggucgccgacgaggucggccugcgcuccgugauugaacaauuuccuggaaagcuggacuucgugcucgucgacgggggauguguccugucgcacggacauaagcagcucaugugccucgcacgguccgugcucuccaaggccaagauucugcugcuggacgaaccuucggcccaccuggauccggucaccuaccagaucaucaggaggacccugaagcaggccuuugccgauugcaccgugauucucugcgagcaccgcaucgaggccaugcuggagugccagcaguuccuggucaucgaggagaacaagguccgccaauacgacuccauucaaaagcuccucaacgagcggucgcuguucagacaagcuauuucaccguccgauagagugaagcucuucccgcaucggaacagcucaaagugcaaaucgaagccgcagaucgcagccuugaaggaagagacugaggaagaggugcaggacacccggcuuuaa

SEQ ID NO: 2 - RNA, 4443 nt, Synthetic Oligonucleotide
augcagcgguccccgcucgaaaaggccagugucguguccaaacucuucuucucauggacucggccuauccuuagaaagggguaucggcagaggcuugaguugucugacaucuaccagauccccucgguagauucggcggauaaccucucggagaagcucgaacgggaaugggaccgcgaacucgcgucuaagaaaaacccgaagcucaucaacgcacugagaaggugcuucuucuggcgguucauguucuacgguaucuucuuguaucucggggaggucacaaaagcaguccaaccccuguuguugggucgcauuaucgccucguacgaccccgauaacaaagaagaacggagcaucgcgaucuaccucgggaucggacuguguuugcuuuucaucgucagaacacuuuuguugcauccagcaaucuucggccuccaucacaucgguaugcagaugcgaaucgcuauguuuagcuugaucuacaaaaagacacugaaacucucgucgcggguguuggauaagauuuccaucggucaguuggugucccugcuuaguaauaaccucaacaaauucgaugagggacuggcgcuggcacauuucguguggauugccccguugcaagucgcccuuuugaugggccuuauuugggagcuguugcaggcaucugccuuuuguggccugggauuucugauuguguuggcauuguuucaggcugggcuugggcggaugaugaugaaguaucgcgaccagagagcggguaaaaucucggaaagacucgucaucacuucggaaaugaucgaaaacauccagucggucaaagccuauugcugggaagaagcuauggagaagaugauugaaaaccuccgccaaacugagcugaaacugacccgcaaggcggcguauguccgguauuucaauucgucagcguucuucuuuuccggguucuucguugucuuucucucgguuuugccuuaugccuugauuaaggggauuauccuccgcaagauuuucaccacgauuucguucugcauuguauugcgcauggcagugacacggcaauuuccgugggccgugcagacaugguaugacucgcuuggagcgaucaacaaaauccaagacuucuugcaaaagcaagaguacaagacccuggaguacaaucuuacuacuacggagguaguaauggagaaugugacggcuuuuugggaagaggguuuuggagaacuguuugagaaagcaaagcagaauaacaacaaccgcaagaccucaaauggggacgauucccuguuuuucucgaacuucucccugcucggaacacccguguugaaggacaucaauuucaagauugagaggggacagcuucucgcgguagcgggaagcacuggugcgggaaaaacuagccucuugauggugauuaugggggagcuugagcccagcgaggggaagauuaaacacuccgggcguaucucauucuguagccaguuuucauggaucaugcccggaaccauuaaagagaacaucauuuucggaguauccuaugaugaguaccgauacagaucggucauuaaggcgugccaguuggaagaggacauuucuaaguucgccgagaaggauaacaucgucuugggagaaggggguauuacauugucgggagggcagcgagcgcggaucagccucgcgagagcgguauacaaagaugcagauuuguaucugcuugauucaccguuuggauaccucgacguauugacagaaaaagaaaucuucgagucgugcguguguaaacuuauggcuaauaagacgagaauccuggugacaucaaaaauggaacaccuuaagaaggcggacaagauccugauccuccacgaaggaucguccuacuuuuacggcacuuucucagaguugcaaaacuugcagccggacuucucaagcaaacucauggggugugacucauucgaccaguucagcgcggaacggcggaacucgaucuugacggaaacgcugcaccgauucucgcuugagggugaugccccgguaucguggaccgagacaaagaagcagucguuuaagcagacaggagaauuuggugagaaaagaaagaacaguaucuugaauccuauuaacucaauucgcaaguucucaaucguccagaaaacuccacugcagaugaauggaauugaagaggauucggacgaaccccuggagcgcaggcuuagccucgugccggauucagagcaaggggaggccauucuuccccggauuucggugauuucaaccggaccuacacuucaggcgaggcgaaggcaauccgugcucaaccucaugacgcauucgguaaaccaggggcaaaacauucaccgcaaaacgacggccucaacgagaaaagugucacuugcaccccaggcgaauuugacugaacucgacaucuacagccguaggcuuucgcaagaaaccggacuugagaucagcgaagaaaucaaugaagaagauuugaaagaguguuucuuugaugacauggaaucaaucccagcggugacaacguggaacacauacuugcguuacaucacggugcacaaguccuugauuuucguccucaucuggugucucgugaucuuucucgcugaggucgcagcgucacuugugguccucuggcugcuugguaauacgcccuugcaagacaaaggcaauucuacacacucaagaaacaauuccuaugccgugauuaucacuucuacaagcucguauuacguguuuuacaucuacguaggaguggccgacacucugcucgcgauggguuucuuccgaggacucccacucguucacacgcuuaucacugucuccaagauucuccaccauaagaugcuucauagcguacugcaggcucccauguccaccuugaauacgcucaaggcgggagguauuuugaaucgcuucucaaaagauauugcaauuuuggaugaccuucugccccugacgaucuucgacuucauccaguuguugcugaucgugauuggggcuauugcaguagucgcuguccuccagccuuacauuuuugucgcgaccguuccggugaucguggcguuuaucaugcugcgggccuauuucuugcagacgucacagcagcuuaagcaacuggagucugaagggaggucgccuaucuuuacgcaucuugugaccaguuugaagggauuguggacguugcgcgccuuuggcaggcagcccuacuuugaaacacuguuccacaaagcgcugaaucuccauacggcaaauugguuuuuguauuugaguacccuccgaugguuucagaugcgcauugagaugauuuuugugaucuucuuuaucgcggugacuuuuaucuccaucuugaccacgggagagggcgagggacgggucgguauuauccugacacucgccaugaacauuaugagcacuuugcagugggcagugaacagcucgauugauguggauagccugaugagguccguuucgagggucuuuaaguucaucgacaugccgacggagggaaagcccacaaaaaguacgaaacccuauaagaaugggcaauugaguaagguaaugaucaucgagaacagucacgugaagaaggaugacaucuggccuagcgggggucagaugaccgugaaggaccugacggcaaaauacaccgagggagggaacgcaauccuugaaaacaucucguucagcauuagccccggucagcgugugggguugcucgggaggaccgggucaggaaaaucgacguugcugucggccuucuugagacuucugaauacagagggugagauccagaucgacggcguuucgugggauagcaucaccuugcagcaguggcggaaagcguuuggaguaaucccccaaaaggucuuuaucuuuagcggaaccuuccgaaagaaucucgauccuuaugaacaguggucagaucaagagauuuggaaagucgcggacgagguuggccuucggaguguaaucgagcaguuuccgggaaaacucgacuuuguccuuguagaugggggaugcguccugucgcaugggcacaagcagcucaugugccuggcgcgauccguccucucuaaagcgaaaauucuucucuuggaugaaccuucggcccaucuggacccgguaacguaucagaucaucagaaggacacuuaagcaggcguuugccgacugcacggugauucucugugagcaucguaucgaggccaugcucgaaugccagcaauuucuugucaucgaagagaauaagguccgccaguacgacuccauccagaagcugcuuaaugagagaucauuguuccggcaggcgauuucaccauccgauagggugaaacuuuuuccacacagaaauucgucgaagugcaaguccaaaccgcagaucgcggccuugaaagaagagacugaagaagaaguucaagacacgcgucuuuaa

SEQ ID NO: 3 - protein, 1480 aa, Homo sapiens
MQRSPLEKASVVSKLFFSWTRPILRKGYRQRLELSDIYQIPSVDSADNLSEKLEREWDRELASKKNPKLINALRRCFFWRFMFYGIFLYLGEVTKAVQPLLLGRIIASYDPDNKEERSIAIYLGIGLCLLFIVRTLLLHPAIFGLHHIGMQMRIAMFSLIYKKTLKLSSRVLDKISIGQLVSLLSNNLNKFDEGLALAHFVWIAPLQVALLMGLIWELLQASAFCGLGFLIVLALFQAGLGRMMMKYRDQRAGKISERLVITSEMIENIQSVKAYCWEEAMEKMIENLRQTELKLTRKAAYVRYFNSSAFFFSGFFVVFLSVLPYALIKGIILRKIFTTISFCIVLRMAVTRQFPWAVQTWYDSLGAINKIQDFLQKQEYKTLEYNLTTTEVVMENVTAFWEEGFGELFEKAKQNNNNRKTSNGDDSLFFSNFSLLGTPVLKDINFKIERGQLLAVAGSTGAGKTSLLMVIMGELEPSEGKIKHSGRISFCSQFSWIMPGTIKENIIFGVSYDEYRYRSVIKACQLEEDISKFAEKDNIVLGEGGITLSGGQRARISLARAVYKDADLYLLDSPFGYLDVLTEKEIFESCVCKLMANKTRILVTSKMEHLKKADKILILHEGSSYFYGTFSELQNLQPDFSSKLMGCDSFDQFSAERRNSILTETLHRFSLEGDAPVSWTETKKQSFKQTGEFGEKRKNSILNPINSIRKFSIVQKTPLQMNGIEEDSDEPLERRLSLVPDSEQGEAILPRISVISTGPTLQARRRQSVLNLMTHSVNQGQNIHRKTTASTRKVSLAPQANLTELDIYSRRLSQETGLEISEEINEEDLKECFFDDMESIPAVTTWNTYLRYITVHKSLIFVLIWCLVIFLAEVAASLVVLWLLGNTPLQDKGNSTHSRNNSYAVIITSTSSYYVFYIYVGVADTLLAMGFFRGLPLVHTLITVSKILHHKMLHSVLQAPMSTLNTLKAGGILNRFSKDIAILDDLLPLTIFDFIQLLLIVIGAIAVVAVLQPYIFVATVPVIVAFIMLRAYFLQTSQQLKQLESEGRSPIFTHLVTSLKGLWTLRAFGRQPYFETLFHKALNLHTANWFLYLSTLRWFQMRIEMIFVIFFIAVTFISILTTGEGEGRVGIILTLAMNIMSTLQWAVNSSIDVDSLMRSVSRVFKFIDMPTEGKPTKSTKPYKNGQLSKVMIIENSHVKKDDIWPSGGQMTVKDLTAKYTEGGNAILENISFSISPGQRVGLLGRTGSGKSTLLSAFLRLLNTEGEIQIDGVSWDSITLQQWRKAFGVIPQKVFIFSGTFRKNLDPYEQWSDQEIWKVADEVGLRSVIEQFPGKLDFVLVDGGCVLSHGHKQLMCLARSVLSKAKILLLDEPSAHLDPVTYQIIRRTLKQAFADCTVILCEHRIEAMLECQQFLVIEENKVRQYDSIQKLLNERSLFRQAISPSDRVKLFPHRNSSKCKSKPQIAALKEETEEEVQDTRL

SEQ ID NO: 4 - RNA, 140 nt, Synthetic Oligonucleotide
ggacagaucgccuggagacgccauccacgcuguuuugaccuccauagaagacaccgggaccgauccagccuccgcggccgggaacggugcauuggaacgcggauuccccgugccaagagugacucaccguccuugacacg

SEQ ID NO: 5 - RNA, 105 nt, Synthetic Oligonucleotide
cggguggcaucccugugaccccuccccagugccucuccuggcccuggaaguugccacuccagugcccaccagccuuguccuaauaaaauuaaguugcaucaagcu

SEQ ID NO: 6 - RNA, 105 nt, Synthetic Oligonucleotide
ggguggcaucccugugaccccuccccagugccucuccuggcccuggaaguugccacuccagugcccaccagccuuguccuaauaaaauuaaguugcaucaaagcu

SEQ ID NO: 7 - RNA, 4688 nt, Synthetic Oligonucleotide
ggacagaucgccuggagacgccauccacgcuguuuugaccuccauagaagacaccgggaccgauccagccuccgcggccgggaacggugcauuggaacgcggauuccccgugccaagagugacucaccguccuugacacgaugcaacgcucuccucuugaaaaggccucggugguguccaagcucuucuucucguggacuagacccauccugagaaagggguacagacagcgcuuggagcuguccgauaucuaucaaaucccuuccguggacuccgcggacaaccuguccgagaagcucgagagagaaugggacagagaacucgccucaaagaagaacccgaagcugauuaaugcgcuuaggcggugcuuuuucuggcgguucauguucuacggcaucuuccucuaccugggagaggucaccaaggccgugcagccccuguugcugggacggauuauugccuccuacgaccccgacaacaaggaagaaagaagcaucgcuaucuacuugggcaucggucugugccugcuuuucaucguccggacccucuuguugcauccugcuauuuucggccugcaucacauuggcaugcagaugagaauugccauguuuucccugaucuacaagaaaacucugaagcucucgagccgcgugcuugacaagauuuccaucggccagcucgugucccugcucuccaacaaucugaacaaguucgacgagggccucgcccuggcccacuucguguggaucgccccucugcaaguggcgcuucugaugggccugaucugggagcugcugcaagccucggcauucugugggcuuggauuccugaucgugcuggcacuguuccaggccggacuggggcggaugaugaugaaguacagggaccagagagccggaaagauuuccgaacggcuggugaucacuucggaaaugaucgaaaacauccagucagugaaggccuacugcugggaagaggccauggaaaagaugauugaaaaccuccggcaaaccgagcugaagcugacccgcaaggccgcuuacgugcgcuauuucaacucguccgcuuucuucuucuccggguucuucgugguguuucucuccgugcuccccuacgcccugauuaagggaaucauccucaggaagaucuucaccaccauuuccuucuguaucgugcuccgcauggccgugacccggcaguucccaugggccgugcagacuugguacgacucccugggagccauuaacaagauccaggacuuccuucaaaagcaggaguacaagacccucgaguacaaccugacuacuaccgaggucgugauggaaaacgucaccgccuuuugggaggagggauuuggcgaacuguucgagaaggccaagcagaacaacaacaaccgcaagaccucgaacggugacgacucccucuucuuuucaaacuucagccugcucgggacgcccgugcugaaggacauuaacuucaagaucgaaagaggacagcuccuggcgguggccggaucgaccggagccggaaagacuucccugcugauggugaucaugggagagcuugaaccuagcgagggaaagaucaagcacuccggccgcaucagcuucuguagccaguuuuccuggaucaugcccggaaccauuaaggaaaacaucaucuucggcguguccuacgaugaauaccgcuaccgguccgugaucaaagccugccagcuggaagaggauauuucaaaguucgcggagaaagauaacaucgugcugggcgaaggggguauuaccuugucggggggccagcgggcuagaaucucgcuggccagagccguguauaaggacgccgaccuguaucuccuggacucccccuucggauaccuggacguccugaccgaaaaggagaucuucgaaucgugcgugugcaagcugauggcuaacaagacucgcauccucgugaccuccaaaauggagcaccugaagaaggcagacaagauucugauucugcaugagggguccuccuacuuuuacggcaccuucucggaguugcagaacuugcagcccgacuucucaucgaagcugauggguugcgacagcuucgaccaguucuccgccgaaagaaggaacucgauccugacggaaaccuugcaccgcuucucuuuggaaggcgacgccccugugucauggaccgagacuaagaagcagagcuucaagcagaccggggaauucggcgaaaagaggaagaacagcaucuugaaccccauuaacuccauccgcaaguucucaaucgugcaaaagacgccacugcagaugaacggcauugaggaggacuccgacgaaccccuugagaggcgccugucccuggugccggacagcgagcagggagaagccauccugccucggauuuccgugaucuccacugguccgacgcuccaagcccggcggcggcaguccgugcugaaccugaugacccacagcgugaaccagggccaaaacauucaccgcaagacuaccgcauccacccggaaagugucccuggcaccucaagcgaaucuuaccgagcucgacaucuacucccggagacugucgcaggaaaccgggcucgaaauuuccgaagaaaucaacgaggaggaucugaaagagugcuucuucgacgauauggagucgauacccgccgugacgacuuggaacacuuaucugcgguacaucacugugcacaagucauugaucuucgugcugauuuggugccuggugauuuuccuggccgaggucgcggccucacugguggugcucuggcuguugggaaacacgccucugcaagacaagggaaacuccacgcacucgagaaacaacagcuaugccgugauuaucacuuccaccuccucuuauuacguguucuacaucuacgucggaguggcggauacccugcucgcgauggguuucuucagaggacugccgcugguccacaccuugaucaccgucagcaagauucuucaccacaagauguugcauagcgugcugcaggcccccauguccacccucaacacucugaaggccggaggcauucugaacagauucuccaaggacaucgcuauccuggacgaucuccugccgcuuaccaucuuugacuucauccagcugcugcugaucgugauuggagcaaucgcagugguggcggugcugcagccuuacauuuucguggccacugugccggucauuguggcguucaucaugcugcgggccuacuuccuccaaaccagccagcagcugaagcaacuggaauccgagggacgaucccccaucuucacucaccuugugacgucguugaagggacuguggacccuccgggcuuucggacggcagcccuacuucgaaacccucuuccacaaggcccugaaccuccacaccgccaauugguuccuguaccuguccacccugcggugguuccagaugcgcaucgagaugauuuucgucaucuucuucaucgcggucacauucaucagcauccugacuaccggagagggagagggacgggucggaauaauccugacccucgccaugaacauuaugagcacccugcagugggcagugaacagcucgaucgacguggacagccugaugcgaagcgucagccgcguguucaaguucaucgacaugccuacugagggaaaacccacuaaguccacuaagcccuacaaaaauggccagcugagcaaggucaugaucaucgaaaacucccacgugaagaaggacgauauuuggcccuccggaggucaaaugaccgugaaggaccugaccgcaaaguacaccgagggaggaaacgccauucucgaaaacaucagcuucuccauuucgccgggacagcgggucggccuucucgggcggaccgguuccgggaagucaacucugcugucggcuuuccuccggcugcugaauaccgagggggaaauccaaauugacggcgugucuugggauuccauuacucugcagcaguggcggaaggccuucggcgugaucccccagaagguguucaucuucucggguaccuuccggaagaaccuggauccuuacgagcaguggagcgaccaagaaaucuggaaggucgccgacgaggucggccugcgcuccgugauugaacaauuuccuggaaagcuggacuucgugcucgucgacgggggauguguccugucgcacggacauaagcagcucaugugccucgcacgguccgugcucuccaaggccaagauucugcugcuggacgaaccuucggcccaccuggauccggucaccuaccagaucaucaggaggacccugaagcaggccuuugccgauugcaccgugauucucugcgagcaccgcaucgaggccaugcuggagugccagcaguuccuggucaucgaggagaacaagguccgccaauacgacuccauucaaaagcuccucaacgagcggucgcuguucagacaagcuauuucaccguccgauagagugaagcucuucccgcaucggaacagcucaaagugcaaaucgaagccgcagaucgcagccuugaaggaagagacugaggaagaggugcaggacacccggcuuuaacggguggcaucccugugaccccuccccagugccucuccuggcccuggaaguugccacuccagugcccaccagccuuguccuaauaaaauuaaguugcaucaagcu

SEQ ID NO: 8 - RNA, 4688 nt, Synthetic Oligonucleotide
ggacagaucgccuggagacgccauccacgcuguuuugaccuccauagaagacaccgggaccgauccagccuccgcggccgggaacggugcauuggaacgcggauuccccgugccaagagugacucaccguccuugacacgaugcaacgcucuccucuugaaaaggccucggugguguccaagcucuucuucucguggacuagacccauccugagaaagggguacagacagcgcuuggagcuguccgauaucuaucaaaucccuuccguggacuccgcggacaaccuguccgagaagcucgagagagaaugggacagagaacucgccucaaagaagaacccgaagcugauuaaugcgcuuaggcggugcuuuuucuggcgguucauguucuacggcaucuuccucuaccugggagaggucaccaaggccgugcagccccuguugcugggacggauuauugccuccuacgaccccgacaacaaggaagaaagaagcaucgcuaucuacuugggcaucggucugugccugcuuuucaucguccggacccucuuguugcauccugcuauuuucggccugcaucacauuggcaugcagaugagaauugccauguuuucccugaucuacaagaaaacucugaagcucucgagccgcgugcuugacaagauuuccaucggccagcucgugucccugcucuccaacaaucugaacaaguucgacgagggccucgcccuggcccacuucguguggaucgccccucugcaaguggcgcuucugaugggccugaucugggagcugcugcaagccucggcauucugugggcuuggauuccugaucgugcuggcacuguuccaggccggacuggggcggaugaugaugaaguacagggaccagagagccggaaagauuuccgaacggcuggugaucacuucggaaaugaucgaaaacauccagucagugaaggccuacugcugggaagaggccauggaaaagaugauugaaaaccuccggcaaaccgagcugaagcugacccgcaaggccgcuuacgugcgcuauuucaacucguccgcuuucuucuucuccggguucuucgugguguuucucuccgugcuccccuacgcccugauuaagggaaucauccucaggaagaucuucaccaccauuuccuucuguaucgugcuccgcauggccgugacccggcaguucccaugggccgugcagacuugguacgacucccugggagccauuaacaagauccaggacuuccuucaaaagcaggaguacaagacccucgaguacaaccugacuacuaccgaggucgugauggaaaacgucaccgccuuuugggaggagggauuuggcgaacuguucgagaaggccaagcagaacaacaacaaccgcaagaccucgaacggugacgacucccucuucuuuucaaacuucagccugcucgggacgcccgugcugaaggacauuaacuucaagaucgaaagaggacagcuccuggcgguggccggaucgaccggagccggaaagacuucccugcugauggugaucaugggagagcuugaaccuagcgagggaaagaucaagcacuccggccgcaucagcuucuguagccaguuuuccuggaucaugcccggaaccauuaaggaaaacaucaucuucggcguguccuacgaugaauaccgcuaccgguccgugaucaaagccugccagcuggaagaggauauuucaaaguucgcggagaaagauaacaucgugcugggcgaaggggguauuaccuugucggggggccagcgggcuagaaucucgcuggccagagccguguauaaggacgccgaccuguaucuccuggacucccccuucggauaccuggacguccugaccgaaaaggagaucuucgaaucgugcgugugcaagcugauggcuaacaagacucgcauccucgugaccuccaaaauggagcaccugaagaaggcagacaagauucugauucugcaugagggguccuccuacuuuuacggcaccuucucggaguugcagaacuugcagcccgacuucucaucgaagcugauggguugcgacagcuucgaccaguucuccgccgaaagaaggaacucgauccugacggaaaccuugcaccgcuucucuuuggaaggcgacgccccugugucauggaccgagacuaagaagcagagcuucaagcagaccggggaauucggcgaaaagaggaagaacagcaucuugaaccccauuaacuccauccgcaaguucucaaucgugcaaaagacgccacugcagaugaacggcauugaggaggacuccgacgaaccccuugagaggcgccugucccuggugccggacagcgagcagggagaagccauccugccucggauuuccgugaucuccacugguccgacgcuccaagcccggcggcggcaguccgugcugaaccugaugacccacagcgugaaccagggccaaaacauucaccgcaagacuaccgcauccacccggaaagugucccuggcaccucaagcgaaucuuaccgagcucgacaucuacucccggagacugucgcaggaaaccgggcucgaaauuuccgaagaaaucaacgaggaggaucugaaagagugcuucuucgacgauauggagucgauacccgccgugacgacuuggaacacuuaucugcgguacaucacugugcacaagucauugaucuucgugcugauuuggugccuggugauuuuccuggccgaggucgcggccucacugguggugcucuggcuguugggaaacacgccucugcaagacaagggaaacuccacgcacucgagaaacaacagcuaugccgugauuaucacuuccaccuccucuuauuacguguucuacaucuacgucggaguggcggauacccugcucgcgauggguuucuucagaggacugccgcugguccacaccuugaucaccgucagcaagauucuucaccacaagauguugcauagcgugcugcaggcccccauguccacccucaacacucugaaggccggaggcauucugaacagauucuccaaggacaucgcuauccuggacgaucuccugccgcuuaccaucuuugacuucauccagcugcugcugaucgugauuggagcaaucgcagugguggcggugcugcagccuuacauuuucguggccacugugccggucauuguggcguucaucaugcugcgggccuacuuccuccaaaccagccagcagcugaagcaacuggaauccgagggacgaucccccaucuucacucaccuugugacgucguugaagggacuguggacccuccgggcuuucggacggcagcccuacuucgaaacccucuuccacaaggcccugaaccuccacaccgccaauugguuccuguaccuguccacccugcggugguuccagaugcgcaucgagaugauuuucgucaucuucuucaucgcggucacauucaucagcauccugacuaccggagagggagagggacgggucggaauaauccugacccucgccaugaacauuaugagcacccugcagugggcagugaacagcucgaucgacguggacagccugaugcgaagcgucagccgcguguucaaguucaucgacaugccuacugagggaaaacccacuaaguccacuaagcccuacaaaaauggccagcugagcaaggucaugaucaucgaaaacucccacgugaagaaggacgauauuuggcccuccggaggucaaaugaccgugaaggaccugaccgcaaaguacaccgagggaggaaacgccauucucgaaaacaucagcuucuccauuucgccgggacagcgggucggccuucucgggcggaccgguuccgggaagucaacucugcugucggcuuuccuccggcugcugaauaccgagggggaaauccaaauugacggcgugucuugggauuccauuacucugcagcaguggcggaaggccuucggcgugaucccccagaagguguucaucuucucggguaccuuccggaagaaccuggauccuuacgagcaguggagcgaccaagaaaucuggaaggucgccgacgaggucggccugcgcuccgugauugaacaauuuccuggaaagcuggacuucgugcucgucgacgggggauguguccugucgcacggacauaagcagcucaugugccucgcacgguccgugcucuccaaggccaagauucugcugcuggacgaaccuucggcccaccuggauccggucaccuaccagaucaucaggaggacccugaagcaggccuuugccgauugcaccgugauucucugcgagcaccgcaucgaggccaugcuggagugccagcaguuccuggucaucgaggagaacaagguccgccaauacgacuccauucaaaagcuccucaacgagcggucgcuguucagacaagcuauuucaccguccgauagagugaagcucuucccgcaucggaacagcucaaagugcaaaucgaagccgcagaucgcagccuugaaggaagagacugaggaagaggugcaggacacccggcuuuaaggguggcaucccugugaccccuccccagugccucuccuggcccuggaaguugccacuccagugcccaccagccuuguccuaauaaaauuaaguugcaucaaagcu

SEQ ID NO: 9 - protein, 874 aa, Bacteriophage SP6
MQDLHAIQLQLEEEMFNGGIRRFEADQQRQIAAGSESDTAWNRRLLSELIAPMAEGIQAYKEEYEGKKGRAPRALAFLQCVENEVAAYITMKVVMDMLNTDATLQAIAMSVAERIEDQVRFSKLEGHAAKYFEKVKKSLKASRTKSYRHAHNVAVVAEKSVAEKDADFDRWEAWPKETQLQIGTTLLEILEGSVFYNGEPVFMRAMRTYGGKTIYYLQTSESVGQWISAFKEHVAQLSPAYAPCVIPPRPWRTPFNGGFHTEKVASRIRLVKGNREHVRKLTQKQMPKVYKAINALQNTQWQINKDVLAVIEEVIRLDLGYGVPSFKPLIDKENKPANPVPVEFQHLRGRELKEMLSPEQWQQFINWKGECARLYTAETKRGSKSAAVVRMVGQARKYSAFESIYFVYAMDSRSRVYVQSSTLSPQSNDLGKALLRFTEGRPVNGVEALKWFCINGANLWGWDKKTFDVRVSNVLDEEFQDMCRDIAADPLTFTQWAKADAPYEFLAWCFEYAQYLDLVDEGRADEFRTHLPVHQDGSCSGIQHYSAMLRDEVGAKAVNLKPSDAPQDIYGAVAQVVIKKNALYMDADDATTFTSGSVTLSGTELRAMASAWDSIGITRSLTKKPVMTLPYGSTRLTCRESVIDYIVDLEEKEAQKAVAEGRTANKVHPFEDDRQDYLTPGAAYNYMTALIWPSISEVVKAPIVAMKMIRQLARFAAKRNEGLMYTLPTGFILEQKIMATEMLRVRTCLMGDIKMSLQVETDIVDEAAMMGAAAPNFVHGHDASHLILTVCELVDKGVTSIAVIHDSFGTHADNTLTLRVALKGQMVAMYIDGNALQKLLEEHEVRWMVDTGIEVPEQGEFDLNEIMDSEYVFA

SEQ ID NO: 10 - DNA, 18 bp, Synthetic Oligonucleotide
atttaggtgacactatag

SEQ ID NO: 11 - DNA, 23 bp, Synthetic Oligonucleotide
atttaggggacactatagaagag

SEQ ID NO: 12 - DNA, 22 bp, Synthetic Oligonucleotide
atttaggggacactatagaagg

SEQ ID NO: 13 - DNA, 23 bp, Synthetic Oligonucleotide
atttaggggacactatagaaggg

SEQ ID NO: 14 - DNA, 20 bp, Synthetic Oligonucleotide
atttaggtgacactatagaa

SEQ ID NO: 15 - DNA, 22 bp, Synthetic Oligonucleotide
atttaggtgacactatagaaga

SEQ ID NO: 16 - DNA, 23 bp, Synthetic Oligonucleotide
atttaggtgacactatagaagag

SEQ ID NO: 17 - DNA, 22 bp, Synthetic Oligonucleotide
atttaggtgacactatagaagg

SEQ ID NO: 18 - DNA, 23 bp, Synthetic Oligonucleotide
atttaggtgacactatagaaggg

SEQ ID NO: 19 - DNA, 23 bp, Synthetic Oligonucleotide
  misc_feature (22)..(22): n is a, c, g, or t
atttaggtgacactatagaagng

SEQ ID NO: 20 - DNA, 24 bp, Synthetic Oligonucleotide
catacgatttaggtgacactatag

SEQ ID NO: 21 - DNA, 4443 bp, Synthetic Oligonucleotide
atgcagaggagcccactggagaaagcctccgtggtgagtaaactcttttttagttggaccagacccatcctgcgaaaaggatacaggcagcgcctcgagttgtcagatatctaccagattccttctgtggactcagctgacaatttgagtgagaagctggagcgggagtgggatagagagctggcgagcaaaaaaaaccccaagcttatcaatgctctgcgccgctgctttttctggaggttcatgttttatgggatcttcctgtacctgggggaggtcaccaaagctgttcagccgctccttcttggccgcatcatcgccagctatgaccctgataataaagaagaaaggtctattgctatttatctgggaattggcctctgcttgctcttcatcgtccgcacccttctgctgcaccctgccatttttggccttcaccacatcggcatgcaaatgagaattgccatgttctccctcatttacaaaaagaccctgaaactttcctcaagagtgttagataaaatatccattggtcagctggtcagcctgctgtccaacaatcttaacaaatttgatgaaggcttggcgctggcccacttcgtgtggattgcacctctgcaggtggccctgttgatgggacttatatgggagctgcttcaagcctctgctttctgtgggctgggctttttgattgtactggcactttttcaggctgggctcggaagaatgatgatgaaatacagagatcagcgggccgggaagatatcagagcgacttgtgatcaccagtgaaatgattgaaaatattcagagcgtgaaagcctactgctgggaagaagccatggagaagatgattgagaacctgaggcagacagagctcaagctcactcggaaggctgcttatgttcgctatttcaacagcagcgccttcttcttcagtggcttctttgttgtcttcctgtctgttctgccatatgcactgataaaaggcattattttacgaaagatcttcaccaccatcagtttttgcatcgttctcaggatggccgtcacaagacagttcccctgggctgtgcagacctggtacgattccttgggggccatcaacaagattcaagatttcttgcaaaaacaagaatataaaactttagaatacaacctcaccaccactgaagtggtcatggaaaatgtgacagccttttgggaggagggttttggagaattgttcgagaaggcaaagcagaataacaacaacaggaagacgagcaatggggacgactctctcttcttcagcaacttttcactgctcgggacccctgtgttgaaagatataaacttcaagatcgagaggggccagctcttggctgtggcaggctccactggagctggtaaaacatctcttctcatggtgatcatgggggaactggagccttccgaaggaaaaatcaagcacagtgggagaatctcattctgcagccagttttcctggatcatgcccggcaccattaaggaaaacatcatatttggagtgtcctatgatgagtaccgctaccggtcagtcatcaaagcctgtcagttggaggaggacatctccaagtttgcagagaaagacaacattgtgcttggagaggggggtatcactctttctggaggacaaagagccaggatctctttggcccgggcagtctacaaggatgcagacctctacttgttggacagtcccttcggctacctcgacgtgctgactgaaaaagaaatttttgaaagctgtgtgtgcaaactgatggcaaacaagaccaggattcttgtcaccagcaagatggaacatctgaagaaagcggacaaaattctgattctgcatgaagggagctcctacttctatggaacatttagcgagcttcagaacctacagccagacttctcctccaaattaatgggctgtgactccttcgaccagttctctgcagaaagaagaaactctatactcacagagaccctccaccgcttctcccttgagggagatgccccagtttcttggacagaaaccaagaagcagtcctttaagcagactggcgagtttggtgaaaagaggaaaaattcaattctcaatccaattaacagtattcgcaagttcagcattgtccagaagacacccctccagatgaatggcatcgaagaagatagtgacgagccgctggagagacggctgagtctggtgccagattcagaacagggggaggccatcctgccccggatcagcgtcatttccacaggccccacattacaagcacggcgccggcagagtgttttaaatctcatgacccattcagtgaaccagggccaaaatatccacaggaagactacagcttctacccggaaagtgtctctggcccctcaggccaatctgaccgagctggacatctacagcaggaggctctcccaggaaacagggctggaaatatctgaagagattaatgaagaggatcttaaagagtgcttctttgatgacatggagagcatccccgcggtgaccacatggaacacctaccttagatatattactgtccacaagagcctcatatttgtcctcatctggtgcctggttattttcctcgctgaggtggcggccagtcttgttgtgctctggctgctgggcaacactcctctccaggacaagggcaatagtactcacagcagaaataattcttatgccgtcatcattacaagcacctccagctactacgtgttctacatctatgtgggcgtggctgacaccctcctggccatgggtttcttccggggcctgcctttggtgcacaccctcatcacagtgtcaaaaattctgcaccataaaatgcttcattctgtcctgcaggcacccatgagcactttgaacacattgaaggctggcggcatcctcaacagattttctaaagatattgctatcctggatgatctcctccccctgacaatctttgactttatccagcttctgctgatcgtgattggagccatagcagtggttgctgtcctgcagccctacatttttgtggccaccgtgcccgtgattgttgcctttattatgctcagagcttacttcctgcaaacttctcaacagctcaaacagctagaatctgagggccggagccccatttttacccacctggtgacttccctgaagggactgtggactctgagagcattcgggcgacagccttactttgagacactgttccacaaggccctgaacttgcacactgccaactggtttctttacctgagcacactccgctggttccagatgcggatagagatgatcttcgtcatcttttttatagctgtaaccttcatttctatccttacaacaggagaaggagagggcagggtgggaatcatcctcacgctggctatgaacataatgtccaccttgcagtgggccgtgaattccagtatagatgtggattctctaatgaggagtgtctcccgggtgtttaaattcattgatatgcctactgaggggaaacccaccaagtcaacaaaaccttataagaatggacagctgagcaaggtgatgataattgagaacagccacgtgaagaaggatgacatttggcccagcgggggccagatgactgtgaaggacctgacggccaagtacaccgaaggtggaaatgccattttggaaaacatcagcttctcaatctctcctgggcagagagttggattgctgggtcgcacgggcagcggcaaatcaaccctgctcagtgccttccttcggctcctgaatacagaaggcgaaatccaaattgacggggtgagctgggacagcatcaccctgcagcagtggagaaaagcatttggggtcattccacagaaagttttcatcttctctggcactttcagaaagaacctggacccctatgagcagtggagcgaccaggagatctggaaggttgcagatgaagttggcctgcggagtgtgatagaacaatttcctggcaagctggattttgtgctggtagatggaggctgcgtgctgtcccacggccacaaacagctgatgtgcctcgcccgctccgttctttcaaaggccaaaatcttgcttttggatgagcccagtgctcacctcgacccagtgacctatcagataatccgcaggaccttaaagcaagcttttgccgactgcaccgtcatactgtgtgagcaccggattgaagcaatgctggaatgccagcagtttctggtgatcgaggagaataaggtccggcagtacgacagcatccagaagttgttgaatgagcgcagccttttccgccaggccatctccccatctgacagagtcaagctgtttccacataggaactcctctaagtgcaagtccaagccccagatcgctgccctcaaggaggaaactgaggaagaggtgcaggatacccgcctgtga

SEQ ID NO: 22 - DNA, 4443 bp, Synthetic Oligonucleotide
atgcagaggagcccactggagaaagcctccgtggtgagtaaactcttttttagttggaccagacccatcctgcgaaaaggatacaggcagcgcctcgagttgtctgatatctaccagattccttctgtggactcagctgacaatttgagtgagaagctggagcgggagtgggatagagagctggcgagcaaaaaaaaccccaagcttatcaatgctctgcgccgctgctttttctggaggttcatgttttatgggatcttcctgtacctgggggaggtcaccaaagctgttcagccgctccttcttggccgcatcatcgccagctatgaccctgataataaagaagaaaggtctattgctatttatctgggaattggcctctgcttgctcttcatcgtccgcacccttctgctgcaccctgccatttttggccttcaccacatcggcatgcaaatgagaattgccatgttctccctcatttacaaaaagaccctgaaactttcctcaagagtgttagataaaatatccattggtcagctggtcagcctgctgtccaacaatcttaacaaatttgatgaaggcttggcgctggcccacttcgtgtggattgcacctctgcaggtggccctgttgatgggacttatatgggagctgcttcaagcctctgctttctgtgggctgggctttttgattgtactggcactttttcaggctgggctcggaagaatgatgatgaaatacagagatcagcgggccgggaagatttcagagcgacttgtgatcaccagtgaaatgattgaaaatattcagagcgtgaaagcctactgctgggaagaagccatggagaagatgattgagaacctgaggcagacagagctcaagctcactcggaaggctgcttatgttcgctatttcaacagcagcgccttcttcttcagtggcttctttgttgtcttcctgtctgttctgccatatgcactgataaaaggcattattttacgaaagatcttcaccaccatcagtttttgcatcgttctcaggatggccgtcacaagacagttcccctgggctgtgcagacctggtacgattccttgggggccatcaacaagattcaagatttcttgcaaaaacaagaatataaaactttagaatacaacctcaccaccactgaagtggtcatggaaaatgtgacagccttttgggaggagggttttggagaattgttcgagaaggcaaagcagaataacaacaacaggaagacgagcaatggggacgactctctcttcttcagcaacttttcactgctcgggacccctgtgttgaaagatataaacttcaagatcgagaggggccagctcttggctgtggcaggctccactggagctggtaaaacatctcttctcatggtgatcatgggggaactggagccttccgaaggaaaaatcaagcacagtgggagaatctcattctgcagccagttttcctggatcatgcccggcaccattaaggaaaacatcatatttggagtgtcctatgatgagtaccgctaccggtcagtcatcaaagcctgtcagttggaggaggacatctccaagtttgcagagaaagacaacattgtgcttggagaggggggtatcactctttctggaggacaaagagccaggatctctttggcccgggcagtctacaaggatgcagacctctacttgttggacagtcccttcggctacctcgacgtgctgactgaaaaagaaatttttgaaagctgtgtgtgcaaactgatggcaaacaagaccaggattcttgtcaccagcaagatggaacatctgaagaaagcggacaaaattctgattctgcatgaagggagctcctacttctatggaacatttagcgagcttcagaacctacagccagacttctcctccaaattaatgggctgtgactccttcgaccagttctctgcagaaagaagaaactctatactcacagagaccctccaccgcttctcccttgagggagatgccccagtttcttggacagaaaccaagaagcagtcctttaagcagactggcgagtttggtgaaaagaggaaaaattcaattctcaatccaattaacagtattcgcaagttcagcattgtccagaagacacccctccagatgaatggcatcgaagaagatagtgacgagccgctggagagacggctgagtctggtgccagattcagaacagggggaggccatcctgccccggatcagcgtcatttccacaggccccacattacaagcacggcgccggcagagtgttttaaatctcatgacccattcagtgaaccagggccaaaatatccacaggaagactacagcttctacccggaaagtgtctctggcccctcaggccaatctgaccgagctggacatctacagcaggaggctctcccaggaaacagggctggaaatatctgaagagattaatgaagaggatcttaaagagtgcttctttgatgacatggagagcatccccgcggtgaccacatggaacacctaccttagatatattactgtccacaagagcctcatatttgtcctcatctggtgcctggttattttcctcgctgaggtggcggccagtcttgttgtgctctggctgctgggcaacactcctctccaggacaagggcaatagtactcacagcagaaataattcttatgccgtcatcattacaagcacctccagctactacgtgttctacatctatgtgggcgtggctgacaccctcctggccatgggtttcttccggggcctgcctttggtgcacaccctcatcacagtgtcaaaaattctgcaccataaaatgcttcattctgtcctgcaggcacccatgagcactttgaacacattgaaggctggcggcatcctcaacagattttctaaagatattgctatcctggatgatctcctccccctgacaatctttgactttatccagcttctgctgatcgtgattggagccatagcagtggttgctgtcctgcagccctacatttttgtggccaccgtgcccgtgattgttgcctttattatgctcagagcttacttcctgcaaacttctcaacagctcaaacagctagaatctgagggccggagccccatttttacccacctggtgacttccctgaagggactgtggactctgagagcattcgggcgacagccttactttgagacactgttccacaaggccctgaacttgcacactgccaactggtttctttacctgagcacactccgctggttccagatgcggatagagatgatcttcgtcatcttttttatagctgtaaccttcatttctatccttacaacaggagaaggagagggcagggtgggaatcatcctcacgctggctatgaacataatgtccaccttgcagtgggccgtgaattccagtatagatgtggattctctaatgaggagtgtctcccgggtgtttaaattcattgatatgcctactgaggggaaacccaccaagtcaacaaaaccttataagaatggacagctgagcaaggtgatgataattgagaacagccacgtgaagaaggatgacatttggcccagcgggggccagatgactgtgaaggacctgacggccaagtacaccgaaggtggaaatgccattttggaaaacatcagcttctcaatctctcctgggcagagagttggattgctgggtcgcacgggcagcggcaaatcaaccctgctcagtgccttccttcggctcctgaatacagaaggcgaaatccaaattgacggggtgagctgggacagcatcaccctgcagcagtggagaaaagcatttggggtcattccacagaaagttttcatcttctctggcactttcagaaagaacctggacccctatgagcagtggagcgaccaggagatctggaaggttgcagatgaagttggcctgcggagtgtgatagaacaatttcctggcaagctggattttgtgctggtagatggaggctgcgtgctgtcccacggccacaaacagctgatgtgcctcgcccgctccgttctttcaaaggccaaaatcttgcttttggatgagcccagtgctcaccttgacccagtgacctatcagataatccgcaggaccttaaagcaagcttttgccgactgcaccgtcatactgtgtgagcaccggattgaagcaatgctggaatgccagcagtttctggtgatcgaggagaataaggtccggcagtacgacagcatccagaagttgttgaatgagcgcagccttttccgccaggccatctccccatctgacagagtcaagctgtttccacataggaactcctctaagtgcaagtccaagccccagatcgctgccctcaaggaggaaactgaggaagaggtgcaggatacccgcctgtga

SEQ ID NO: 23 - DNA, 4443 bp, Synthetic Oligonucleotide
atgcagaggagcccactggagaaagcctccgtggtgagtaaactcttttttagttggaccagacccatcctgcgaaaaggatacaggcagcgcctcgagttgtcagatatctaccagattccttctgtggactcagctgacaatttgagtgagaagctggagcgggagtgggatagagagctggcgagcaaaaaaaaccccaagcttatcaatgctctgcgccgctgctttttctggaggttcatgttttatgggatcttcctgtacctgggggaggtcaccaaagctgttcagccgctccttcttggccgcatcatcgccagctatgaccctgataataaagaagaaaggtctattgctatttatctgggaattggcctctgcttgctcttcatcgtccgcacccttctgctgcaccctgccatttttggccttcaccacatcggcatgcaaatgagaattgccatgttctccctcatttacaaaaagaccctgaaactttcctcaagagtgttagataaaatatccattggtcagctggtcagcctgctgtccaacaatcttaacaaatttgatgaaggcttggcgctggcccacttcgtgtggattgcacctctgcaggtggccctgttgatgggacttatatgggagctgcttcaagcctctgctttctgtgggctgggctttttgattgtactggcactttttcaggctgggctcggaagaatgatgatgaaatacagagatcagcgggccgggaagatatcagagcgacttgtgatcaccagtgaaatgattgaaaatattcagagcgtgaaagcctactgctgggaagaagccatggagaagatgattgagaacctgaggcagacagagctcaagctcactcggaaggctgcttatgttcgctatttcaacagcagcgccttcttcttcagtggcttctttgttgtcttcctgtctgttctgccatatgcactgataaaaggcattattttacgaaagatcttcaccaccatcagtttttgcatcgttctcaggatggccgtcacaagacagttcccctgggctgtgcagacctggtacgattccttgggggccatcaacaagattcaagatttcttgcaaaaacaagaatataaaactttagaatacaacctcaccaccactgaagtggtcatggaaaatgtgacagccttttgggaggagggttttggagaattgttcgagaaggcaaagcagaataacaacaacaggaagacgagcaatggggacgactctctcttcttcagcaacttttcactgctcgggacccctgtgttgaaagatataaacttcaagatcgagaggggccagctcttggctgtggcaggctccactggagctggtaaaacatctcttctcatggtgatcatgggggaactggagccttccgaaggaaaaatcaagcacagtgggagaatctcattctgcagccagttttcctggatcatgcccggcaccattaaggaaaacatcatatttggagtgtcctatgatgagtaccgctaccggtcagtcatcaaagcctgtcagttggaggaggacatctccaagtttgcagagaaagacaacattgtgcttggagaggggggtatcactctttctggaggacaaagagccaggatctctttggcccgggcagtctacaaggatgcagacctctacttgttggacagtcccttcggctacctcgacgtgctgactgaaaaagaaatttttgaaagctgtgtgtgcaaactgatggcaaacaagaccaggattcttgtcaccagcaagatggaacatctgaagaaagcggacaaaattctgattctgcatgaagggagctcctacttctatggaacatttagcgagcttcagaacctacagccagacttctcctccaaattaatgggctgtgactccttcgaccagttctctgcagaaagaagaaactctatactcacagagaccctccaccgcttctcccttgagggagatgccccagtttcttggacagaaaccaagaagcagtcctttaagcagactggcgagtttggtgaaaagaggaaaaattcaattctcaatccaattaacagtattcgcaagttcagcattgtccagaagacacccctccagatgaatggcatcgaagaagatagtgacgagccgctggagagacggctgagtctggtgccagattcagaacagggggaggccatcctgccccggatcagcgtcatttccacaggccccacattacaagcacggcgccggcagagtgttttaaatctcatgacccattcagtgaaccagggccaaaatatccacaggaagactacagcttctacccggaaagtgtctctggcccctcaggccaatctgaccgagctggacatctacagcaggaggctctcccaggaaacagggcttgaaatatctgaagagattaatgaagaggatcttaaagagtgcttctttgatgacatggagagcatccccgcggtgaccacatggaacacctaccttagatatattactgtccacaagagcctcatatttgtcctcatctggtgcctggttattttcctcgctgaggtggcggccagtcttgttgtgctctggctgctgggcaacactcctctccaggacaagggcaatagtacacacagcagaaataattcttatgccgtcatcattacaagcacctccagctactacgtgttctacatctatgtgggcgtggctgacaccctcctggccatgggtttcttccggggcctgcctttggtgcacaccctcatcacagtgtcaaaaattctgcaccataaaatgcttcattctgtcctgcaggcacccatgagcactttgaacacattgaaggctggcggcatcctcaacagattttctaaagatattgctatcctggatgatctcctccccctgacaatctttgactttatccagcttctgctgatcgtgattggagccatagcagtggttgctgtcctgcagccctacatttttgtggccaccgtgcccgtgattgttgcctttattatgctcagagcttacttcctgcaaacttctcaacagctcaaacagctagaatctgagggccggagccccatttttacccacctggtgacttccctgaagggactgtggactctgagagcattcgggcgacagccttactttgagacactgttccacaaggccctgaacttgcacactgccaactggtttctttacctgagcacactccgctggttccagatgcggatagagatgatcttcgtcatcttttttatagctgtaaccttcatttctatccttacaacaggagaaggagagggcagggtgggaatcatcctcacgctggctatgaacataatgtccaccttgcagtgggccgtgaattccagtatagatgtggattctctaatgaggagtgtctcccgggtgtttaaattcattgatatgcctactgaggggaaacccaccaagtcaacaaaaccttataagaatggacagctgagcaaggtgatgataattgagaacagccacgtgaagaaggatgacatttggcccagcgggggccagatgactgtgaaggacctgacggccaagtacaccgaaggtggaaatgccattttggaaaacatcagcttctcaatctctcctgggcagagagttggattgctgggtcgcacgggcagcggcaaatcaaccctgctcagtgccttccttcggctcctgaatacagaaggcgaaatccaaattgacggggtgagctgggacagcatcaccctgcagcagtggagaaaagcatttggggtcattccacagaaagttttcatcttctctggcactttcagaaagaacctggacccctatgagcagtggagcgaccaggagatctggaaggttgcagatgaagttggcctgcggagtgtgatagaacaatttcctggcaagctggattttgtgctggtagatggaggctgcgtgctgtcccacggccacaaacagctgatgtgcctcgcccgctccgttctttcaaaggccaaaatcttgcttttggatgagcccagtgctcaccttgacccagtgacctatcagataatccgcaggaccttaaagcaagcttttgccgactgcaccgtcatactgtgtgagcaccggattgaagcaatgctggaatgccagcagtttctggtgatcgaggagaataaggtccggcagtacgacagcatccagaagttgttgaatgagcgcagccttttccgccaggccatctccccatctgacagagtcaagctgtttccacataggaactcctctaagtgcaagtccaagccccagatcgctgccctcaaggaggaaactgaggaagaggtgcaggatacccgcctgtga

SEQ ID NO: 24 - DNA, 4443 bp, Synthetic Oligonucleotide
atgcagaggagcccactggagaaagcctccgtggtgagtaaactcttttttagttggaccagacccatcctgcgaaaaggatacaggcagcgcctcgagttgtcagatatctaccagattccttctgtggactcagctgacaatttgagtgagaagctggagcgggagtgggatagagagctggcgagcaaaaaaaaccccaagcttatcaatgctctgcgccgctgctttttctggaggttcatgttttatgggatcttcctgtacctgggggaggtcaccaaagctgttcagccgctccttcttggccgcatcatcgccagctatgaccctgataataaagaagaaaggtctattgctatttatctgggaattggcctctgcttgctcttcatcgtccgcacccttctgctgcaccctgccatttttggccttcaccacatcggcatgcaaatgagaattgccatgttctccctcatttacaaaaagaccctgaaactttcctcaagagtgttagataaaatatccattggtcagctggtcagcctgctgtccaacaatcttaacaaatttgatgaaggcttggcgctggcccacttcgtgtggattgcacctctgcaggtggccctgttgatgggacttatatgggagctgcttcaagcctctgctttctgtgggctgggctttttgattgtactggcactttttcaggctgggctcggaagaatgatgatgaaatacagagatcagcgggccgggaagatatcagagcgacttgtgatcaccagtgaaatgattgaaaatattcagagcgtgaaagcctactgctgggaagaagccatggagaagatgattgagaacctgaggcagacagagctcaagctcactcggaaggctgcttatgttcgctatttcaacagcagcgccttcttcttcagtggcttctttgttgtcttcctgtctgttctgccatatgcactgataaaaggcattattttacgaaagatcttcaccaccatcagtttttgcatcgttctcaggatggccgtcacaagacagttcccctgggctgtgcagacctggtacgattccttgggggccatcaacaagattcaagatttcttgcaaaaacaagaatataaaactttagaatacaacctcaccaccactgaagtggtcatggaaaatgtgacagccttttgggaggagggttttggagaattgttcgagaaggcaaagcagaataacaacaacaggaagacgagcaatggggacgactctctcttcttcagcaacttttcactgctcgggacccctgtgttgaaagatataaacttcaagatcgagaggggccagctcttggctgtggcaggctccactggagctggtaaaacatctcttctcatggtgatcatgggggaactggagccttccgaaggaaaaatcaagcacagtgggagaatctcattctgcagccagttttcctggatcatgcccggcaccattaaggaaaacatcatatttggagtgtcctatgatgagtaccgctaccggtcagtcatcaaagcctgtcagttggaggaggacatctccaagtttgcagagaaagacaacattgtgcttggagaggggggtatcactctttctggaggacaaagagccaggatctctttggcccgggcagtctacaaggatgcagacctctacttgttggacagtcccttcggctacctcgacgtgctgactgaaaaagaaatttttgaaagctgtgtgtgcaaactgatggcaaacaagaccaggattcttgtcaccagcaagatggaacatctgaagaaagcggacaaaattctgattctgcatgaagggagctcctacttctatggaacatttagcgagcttcagaacctacagccagacttctcctccaaattaatgggctgtgactccttcgaccagttctctgcagaaagaagaaactctatactcacagagaccctccaccgcttctcccttgagggagatgccccagtttcttggacagaaaccaagaagcagtcctttaagcagactggcgagtttggtgaaaagaggaaaaattcaattctcaatccaattaacagtattcgcaagttcagcattgtccagaagacacccctccagatgaatggcatcgaagaagatagtgacgagccgctggagagacggctgagtctggtgccagattcagaacagggggaggccatcctgccccggatcagcgtcatttccacaggccccacattacaagcacggcgccggcagagtgttttaaatctcatgacccattcagtgaaccagggccaaaatatccacaggaagactacagcttctacccggaaagtgtctctggcccctcaggccaatctgaccgagctggacatctacagcaggaggctctcccaggaaacagggctggaaatatctgaagagattaatgaagaggatcttaaagagtgcttctttgatgacatggagagcatccccgcggtgaccacatggaacacctaccttagatatattactgtccacaagagcctcatatttgtcctcatctggtgcctggttattttcctcgctgaggtggcggccagtcttgttgtgctctggctgctgggcaacactcctctccaggacaagggcaatagtactcacagcagaaataattcttatgccgtcatcattacaagcacctccagctactacgtgttctacatctatgtgggcgtggctgacaccctcctggccatgggtttcttccggggcctgcctttggtgcacaccctcatcacagtgtcaaaaattctgcaccataaaatgcttcattctgtcctgcaggcacccatgagcactttgaacacattgaaggctggcggcatcctcaacagattttctaaagatattgctatcctggatgatctcctccccctgacaatctttgactttatccagcttctgctgatcgtgattggagccatagcagtggttgctgtcctgcagccctacatttttgtggccaccgtgcccgtgattgttgcctttattatgctcagagcttacttcctgcaaacttctcaacagctcaaacagctagaatctgagggccggagccccatttttacccacctggtgacttccctgaagggactgtggactctgagagcattcgggcgacagccttactttgagacactgttccacaaggccctgaacttgcacactgccaactggtttctttacctgagcacactccgctggttccagatgcggatagagatgatcttcgtcatcttttttatagctgtaaccttcatttctatccttacaacaggagaaggagagggcagggtgggaatcatcctcacgctggctatgaacataatgtccaccttgcagtgggccgtgaattccagtatagatgtggattctctaatgaggagtgtctcccgggtgtttaaattcattgatatgccaactgaggggaaacccaccaagtcaacaaaaccttataagaatggacagctgagcaaggtgatgataattgagaacagccacgtgaagaaggatgacatttggcccagcgggggccagatgactgtgaaggacctgacggccaagtacaccgaaggtggaaatgccattttggaaaacatcagcttctcaatctctcctgggcagagagttggattgctgggtcgcacgggcagcggcaaatcaaccctgctcagtgccttccttcggctcctgaatacagaaggcgaaatccaaattgacggggtgagctgggacagcatcaccctgcagcagtggagaaaagcatttggggtcattccacagaaagttttcatcttctctggcactttcagaaagaacctggacccctatgagcagtggagcgaccaggagatctggaaggttgcagatgaagttggcctgcggagtgtgatagaacaatttcctggcaagctggattttgtgctggtagatggaggctgcgtgctgtcccacggccacaaacagctgatgtgcctcgcccgctccgttctttcaaaggccaaaatcttgcttttggatgagcccagtgctcacctcgacccagtgacctatcagataatccgcaggaccttaaagcaagcttttgccgactgcaccgtcatactgtgtgagcaccggattgaagcaatgctggaatgccagcagtttctggtgatcgaggagaataaggtccggcagtacgacagcatccagaagttgttgaatgagcgcagccttttccgccaggccatctccccatctgacagagtcaagctgtttccacataggaactcctctaagtgcaagtccaagccccagatcgctgccctcaaggaggaaactgaggaagaggtgcaggatacccgcctgtga

SEQ ID NO: 25 - DNA, 4443 bp, Synthetic Oligonucleotide
atgcagaggagcccactggagaaagcctccgtggtgagtaaactcttttttagttggaccagacccatcctgcgaaaaggatacaggcagcgcctcgagttgtcagatatctaccagattccttctgtggactcagctgacaatttgagtgagaagctggagcgggagtgggatagagagctggcgagcaaaaaaaaccccaagcttatcaatgctctgcgccgctgctttttctggaggttcatgttttatgggatcttcctgtacctgggggaggtcaccaaagctgttcagccgctccttcttggccgcatcatcgccagctatgaccctgataataaagaagaaaggtctattgctatttatctgggaattggcctctgcttgctcttcatcgtccgcacccttctgctgcaccctgccatttttggccttcaccacatcggcatgcaaatgagaattgccatgttctccctcatttacaaaaagaccctgaaactttcctcaagagtgttagataaaatatccattggtcagctggtcagcctgctgtccaacaatcttaacaaatttgatgaaggcttggcgctggcccacttcgtgtggattgcacctctgcaggtggccctgttgatgggacttatatgggagctgcttcaagcctctgctttctgtgggctgggctttttgattgtactggcactttttcaggctgggctcggaagaatgatgatgaaatacagagatcagcgggccgggaagatatcagagcgacttgtgatcaccagtgaaatgattgaaaatattcagagcgtgaaagcctactgctgggaagaagccatggagaagatgattgagaacctgaggcagacagagctcaagctcactcggaaggctgcttatgttcgctatttcaacagcagcgccttcttcttcagtggcttctttgttgtcttcctgtctgttctgccatatgcactgataaaaggcattattttacgaaagatcttcaccaccatcagtttttgcatcgttctcaggatggccgtcacaagacagttcccctgggctgtgcagacctggtacgattccttgggggccatcaacaagattcaagatttcttgcaaaaacaagaatataaaactttagaatacaacctcaccaccactgaagtggtcatggaaaatgtgacagccttttgggaggagggttttggagaattgttcgagaaggcaaagcagaataacaacaacaggaagacgagcaatggggacgactctctcttcttcagcaacttttcactgctcgggacccctgtgttgaaagatataaacttcaagatcgagaggggccagctcttggctgtggcaggctccactggagctggtaaaacatctcttctcatggtgatcatgggggaactggagccttccgaaggaaaaatcaagcacagtgggagaatctcattctgcagccagttttcctggatcatgcccggcaccattaaggaaaacatcatatttggagtgtcctatgatgagtaccgctaccggtcagtcatcaaagcctgtcagttggaggaggacatctccaagtttgcagagaaagacaacattgtgcttggagaggggggtatcactctttctggaggacaaagagccaggatctctttggcccgggcagtctacaaggatgcagacctctacttgttggacagtcccttcggctacctcgacgtgctgactgaaaaagaaatttttgaaagctgtgtgtgcaaactgatggcaaacaagaccaggattcttgtcaccagcaagatggaacatctgaagaaagcggacaaaattctgattctgcatgaagggagctcctacttctatggaacatttagcgagcttcagaacctacagccagacttctcctccaaattaatgggctgtgactccttcgaccagttctctgcagaaagaagaaactctatactcacagagaccctccaccgcttctcccttgagggagatgccccagtttcttggacagaaaccaagaagcagtcctttaagcagactggcgagtttggtgaaaagaggaaaaattcaattctcaatcctattaacagtattcgcaagttcagcattgtccagaagacacccctccagatgaatggcatcgaagaagatagtgacgagccgctggagagacggctgagtctggtgccagattcagaacagggggaggccatcctgccccggatcagcgtcatttccacaggccccacattacaagcacggcgccggcagagtgttttaaatctcatgacccattcagtgaaccagggccaaaatatccacaggaagactacagcttctacccggaaagtgtctctggcccctcaggccaatctgaccgagctggacatctacagcaggaggctctcccaggaaacagggcttgaaatatctgaagagattaatgaagaggatcttaaagagtgcttctttgatgacatggagagcatccccgcggtgaccacatggaacacctaccttagatatattactgtccacaagagcctcatatttgtcctcatctggtgcctggttattttcctcgctgaggtggcggccagtcttgttgtgctctggctgctgggcaacactcctctccaggacaagggcaatagtactcacagcagaaataattcttatgccgtcatcattacaagcacctccagctactacgtgttctacatctatgtgggcgtggctgacaccctcctggccatgggtttcttccggggcctgcctttggtgcacaccctcatcacagtgtcaaaaattctgcaccataaaatgcttcattctgtcctgcaggcacccatgagcactttgaacacattgaaggctggcggcatcctcaacagattttctaaagatattgctatcctggatgatctcctccccctgacaatctttgactttatccagcttctgctgatcgtgattggagccatagcagtggttgctgtcctgcagccctacatttttgtggccaccgtgcccgtgattgttgcctttattatgctcagagcttacttcctgcaaacttctcaacagctcaaacagctagaatctgagggccggagccccatttttacccacctggtgacttccctgaagggactgtggactctgagagcattcgggcgacagccttactttgagacactgttccacaaggccctgaacttgcacactgccaactggtttctttacctgagcacactccgctggttccagatgcggatagagatgatcttcgtcatcttttttatagctgtaaccttcatttctatccttacaacaggagaaggagagggcagggtgggaatcatcctcacgctggctatgaacataatgtccaccttgcagtgggccgtgaattccagtatagatgtggattctctaatgaggagtgtctcccgggtgtttaaattcattgatatgcctactgaggggaaacccaccaagtcaacaaaaccttataagaatggacagctgagcaaggtgatgataattgagaacagccacgtgaagaaggatgacatttggcccagcgggggccagatgactgtgaaggacctgacggccaagtacaccgaaggtggaaatgccattttggaaaacatcagcttctcaatctctcctgggcagagagttggattgctgggtcgcacgggcagcggcaaatcaaccctgctcagtgccttccttcggctcctgaatacagaaggcgaaatccaaattgacggggtgagctgggacagcatcaccctgcagcagtggagaaaagcatttggggtcattccacagaaagttttcatcttctctggcactttcagaaagaacctggacccctatgagcagtggagcgaccaggagatctggaaggttgcagatgaagttggcctgcggagtgtgatagaacaatttcctggcaagctggattttgtgctggtagatggaggctgcgtgctgtcccacggccacaaacagctgatgtgcctcgcccgctccgttctttcaaaggccaaaatcttgcttttggatgagcccagtgctcacctcgacccagtgacctatcagataatccgcaggaccttaaagcaagcttttgccgactgcaccgtcatactgtgtgagcaccggattgaagcaatgctggaatgccagcagtttctggtgatcgaggagaataaggtccggcagtacgacagcatccagaagttgttgaatgagcgcagccttttccgccaggccatctccccatctgacagagtcaagctgtttccacataggaactcctctaagtgcaagtccaagccccagatcgctgccctcaaggaggaaactgaggaagaggtgcaggatacccgcctgtga

SEQ ID NO: 26 - DNA, 4443 bp, Synthetic Oligonucleotide
atgcagaggagcccactggagaaagcctccgtggtgagtaaactcttttttagttggaccagacccatcctgcgaaaaggatacaggcagcgcctcgagttgtcagatatctaccagattccttctgtggactcagctgacaatttgagtgagaagctggagcgggagtgggatagagagctggcgagcaaaaaaaaccccaagcttatcaatgctctgcgccgctgctttttctggaggttcatgttttatgggatcttcctgtacctgggggaggtcaccaaagctgttcagccgctccttcttggccgcatcatcgccagctatgaccctgataataaagaagaaaggtctattgctatttatctgggaattggcctctgcttgctcttcatcgtccgcacccttctgctgcaccctgccatttttggccttcaccacatcggcatgcaaatgagaattgccatgttctccctcatttacaaaaagaccctgaaactttcctcaagagtgttagataaaatatccattggtcagctggtcagcctgctgtccaacaatcttaacaaatttgatgaaggcttggcgctggcccacttcgtgtggattgcacctctgcaggtggccctgttgatgggacttatatgggagctgcttcaagcctctgctttctgtgggctgggctttttgattgtactggcactttttcaggctgggctcggaagaatgatgatgaaatacagagatcagcgggccgggaagatttcagagcgacttgtgatcaccagtgaaatgattgaaaatattcagagcgtgaaagcctactgctgggaagaagccatggagaagatgattgagaacctgaggcagacagagctcaagctcactcggaaggctgcttatgttcgctatttcaacagcagcgccttcttcttcagtggcttctttgttgtcttcctgtctgttctgccatatgcactgataaaaggcattattttacgaaagatcttcaccaccatcagtttttgcatcgttctcaggatggccgtcacaagacagttcccctgggctgtgcagacctggtacgattccttgggggccatcaacaagattcaagatttcttgcaaaaacaagaatataaaactttagaatacaacctcaccaccactgaagtggtcatggaaaatgtgacagccttttgggaggagggttttggagaattgttcgagaaggcaaagcagaataacaacaacaggaagacgagcaatggggacgactctctcttcttcagcaacttttcactgctcgggacccctgtgttgaaagatataaacttcaagatcgagaggggccagctcttggctgtggcaggctccactggagctggtaaaacatctcttctcatggtgatcatgggggaactggagccttccgaaggaaaaatcaagcacagtgggagaatctcattctgcagccagttttcctggatcatgcccggcaccattaaggaaaacatcatatttggagtgtcctatgatgagtaccgctaccggtcagtcatcaaagcctgtcagttggaggaggacatctccaagtttgcagagaaagacaacattgtgcttggagaggggggtatcactctttctggaggacaaagagccaggatctctttggcccgggcagtctacaaggatgcagacctctacttgttggacagtcccttcggctacctcgacgtgctgactgaaaaagaaatttttgaaagctgtgtgtgcaaactgatggcaaacaagaccaggattcttgtcaccagcaagatggaacatctgaagaaagcggacaaaattctgattctgcatgaagggagctcctacttctatggaacatttagcgagcttcagaacctacagccagacttctcctccaaattaatgggctgtgactccttcgaccagttctctgcagaaagaagaaactctatactcacagagaccctccaccgcttctcccttgagggagatgccccagtttcttggacagaaaccaagaagcagtcctttaagcagactggcgagtttggtgaaaagaggaaaaattcaattctcaatccaattaacagtattcgcaagttcagcattgtccagaagacacccctccagatgaatggcatcgaagaagatagtgacgagccgctggagagacggctgagtctggtgccagattcagaacagggggaggccatcctgccccggatcagcgtcatttccacaggccccacattacaagcacggcgccggcagagtgttttaaatctcatgacccattcagtgaaccagggccaaaatatccacaggaagactacagcttctacccggaaagtgtctctggcccctcaggccaatctgaccgagctggacatctacagcaggaggctctcccaggaaacagggctggaaatatctgaagagattaatgaagaggatcttaaagagtgcttctttgatgacatggagagcatccccgcggtgaccacatggaacacctaccttagatatattactgtccacaagagcctcatatttgtcctcatctggtgcctggttattttcctcgctgaggtggcggccagtcttgttgtgctctggctgctgggcaacactcctctccaggacaagggcaatagtactcacagcagaaataattcttatgccgtcatcattacaagcacctccagctactacgtgttctacatctatgtgggcgtggctgacaccctcctggccatgggtttcttccggggcctgcctttggtgcacaccctcatcacagtgtcaaaaattctgcaccataaaatgcttcattctgtcctgcaggcacccatgagcactttgaacacattgaaggctggcggcatcctcaacagattttctaaagatattgctatcctggatgatctcctccccctgacaatctttgactttatccagcttctgctgatcgtgattggagccatagcagtggttgctgtcctgcagccctacatttttgtggccaccgtgcccgtgattgttgcctttattatgctcagagcttacttcctgcaaacttctcaacagctcaaacagctagaatctgagggccggagccccatttttacccacctggtgacttccctgaagggactgtggactctgagagcattcgggcgacagccttactttgagacactgttccacaaggccctgaacttgcacactgccaactggtttctttacctgagcacactccgctggttccagatgcggatagagatgatcttcgtcatcttttttatagctgtaaccttcatttctatccttacaacaggagaaggagagggcagggtgggaatcatcctcacgctggctatgaacataatgtccaccttgcagtgggccgtgaattccagtatagatgtggattctctaatgaggagtgtctcccgggtgtttaaattcattgatatgccaactgaggggaaacccaccaagtcaacaaaaccttataagaatggacagctgagcaaggtgatgataattgagaacagccacgtgaagaaggatgacatttggcccagcgggggccagatgactgtgaaggacctgacggccaagtacaccgaaggtggaaatgccattttggaaaacatcagcttctcaatctctcctgggcagagagttggattgctgggtcgcacgggcagcggcaaatcaaccctgctcagtgccttccttcggctcctgaatacagaaggcgaaatccaaattgacggggtgagctgggacagcatcaccctgcagcagtggagaaaagcatttggggtcattccacagaaagttttcatcttctctggcactttcagaaagaacctggacccctatgagcagtggagcgaccaggagatctggaaggttgcagatgaagttggcctgcggagtgtgatagaacaatttcctggcaagctggattttgtgctggtagatggaggctgcgtgctgtcccacggccacaaacagctgatgtgcctcgcccgctccgttctttcaaaggccaaaatcttgcttttggatgagcccagtgctcacctcgacccagtgacctatcagataatccgcaggaccttaaagcaagcttttgccgactgcaccgtcatactgtgtgagcaccggattgaagcaatgctggaatgccagcagtttctggtgatcgaggagaataaggtccggcagtacgacagcatccagaagttgttgaatgagcgcagccttttccgccaggccatctccccatctgacagagtcaagctgtttccacataggaactcctctaagtgcaagtccaagccccagatcgctgccctcaaggaggaaactgaggaagaggtgcaggatacccgcctgtga

SEQ ID NO: 27 - DNA, 4443 bp, Synthetic Oligonucleotide
atgcagaggagcccactggagaaagcctccgtggtgagtaaactcttttttagttggaccagacccatcctgcgaaaaggatacaggcagcgcctcgagttgtctgatatctaccagattccttctgtggactcagctgacaatttgagtgagaagctggagcgggagtgggatagagagctggcgagcaaaaaaaaccccaagcttatcaatgctctgcgccgctgctttttctggaggttcatgttttatgggatcttcctgtacctgggggaggtcaccaaagctgttcagccgctccttcttggccgcatcatcgccagctatgaccctgataataaagaagaaaggtctattgctatttatctgggaattggcctctgcttgctcttcatcgtccgcacccttctgctgcaccctgccatttttggccttcaccacatcggcatgcaaatgagaattgccatgttctccctcatttacaaaaagaccctgaaactttcctcaagagtgttagataaaatatccattggtcagctggtcagcctgctgtccaacaatcttaacaaatttgatgaaggcttggcgctggcccacttcgtgtggattgcacctctgcaggtggccctgttgatgggacttatatgggagctgcttcaagcctctgctttctgtgggctgggctttttgattgtactggcactttttcaggctgggctcggaagaatgatgatgaaatacagagatcagcgggccgggaagatatcagagcgacttgtgatcaccagtgaaatgattgaaaatattcagagcgtgaaagcctactgctgggaagaagccatggagaagatgattgagaacctgaggcagacagagctcaagctcactcggaaggctgcttatgttcgctatttcaacagcagcgccttcttcttcagtggcttctttgttgtcttcctgtctgttctgccatatgcactgataaaaggcattattttacgaaagatcttcaccaccatcagtttttgcatcgttctcaggatggccgtcacaagacagttcccctgggctgtgcagacctggtacgattccttgggggccatcaacaagattcaagatttcttgcaaaaacaagaatataaaactttagaatacaacctcaccaccactgaagtggtcatggaaaatgtgacagccttttgggaggagggttttggagaattgttcgagaaggcaaagcagaataacaacaacaggaagacgagcaatggggacgactctctcttcttcagcaacttttcactgctcgggacccctgtgttgaaagatataaacttcaagatcgagaggggccagctcttggctgtggcaggctccactggagctggtaaaacatctcttctcatggtgatcatgggggaactggagccttccgaaggaaaaatcaagcacagtgggagaatctcattctgcagccagttttcctggatcatgcccggcaccattaaggaaaacatcatatttggagtgtcctatgatgagtaccgctaccggtccgtcatcaaagcctgtcagttggaggaggacatctccaagtttgcagagaaagacaacattgtgcttggagaggggggtatcactctttctggaggacaaagagccaggatctctttggcccgggcagtctacaaggatgcagacctctacttgttggacagtcccttcggctacctcgacgtgctgactgaaaaagaaatttttgaaagctgtgtgtgcaaactgatggcaaacaagaccaggattcttgtcaccagcaagatggaacatctgaagaaagcggacaaaattctgattctgcatgaagggagctcctacttctatggaacatttagcgagcttcagaacctacagccagacttctcctccaaattaatgggctgtgactccttcgaccagttctctgcagaaagaagaaactctatactcacagagaccctccaccgcttctcccttgagggagatgccccagtttcttggacagaaaccaagaagcagtcctttaagcagactggcgagtttggtgaaaagaggaaaaattcaattctcaatccaattaacagtattcgcaagttcagcattgtccagaagacacccctccagatgaatggcatcgaagaagatagtgacgagccgctggagagacggctgagtctggtgccagattcagaacagggggaggccatcctgccccggatcagcgtcatttccacaggccccacattacaagcacggcgccggcagagtgttttaaatctcatgacccattcagtgaaccagggccaaaatatccacaggaagactacagcttctacccggaaagtgtctctggcccctcaggccaatctgaccgagctggacatctacagcaggaggctctcccaggaaacagggcttgaaatatctgaagagattaatgaagaggatcttaaagagtgcttctttgatgacatggagagcatccccgcggtgaccacatggaacacctaccttagatatattactgtccacaagagcctcatatttgtcctcatctggtgcctggttattttcctcgctgaggtggcggccagtcttgttgtgctctggctgctgggcaacactcctctccaggacaagggcaatagtactcacagcagaaataattcttatgccgtcatcattacaagcacctccagctactacgtgttctacatctatgtgggcgtggctgacaccctcctggccatgggtttcttccggggcctgcctttggtgcacaccctcatcacagtgtcaaaaattctgcaccataaaatgcttcattctgtcctgcaggcacccatgagcactttgaacacattgaaggctggcggcatcctcaacagattttctaaagatattgctatcctggatgatctcctccccctgacaatctttgactttatccagcttctgctgatcgtgattggagccatagcagtggttgctgtcctgcagccctacatttttgtggccaccgtgcccgtgattgttgcctttattatgctcagagcttacttcctgcaaacttctcaacagctcaaacagctagaatctgagggccggagccccatttttacccacctggtgacttccctgaagggactgtggactctgagagcattcgggcgacagccttactttgagacactgttccacaaggccctgaacttgcacactgccaactggtttctttacctgagcacactccgctggttccagatgcggatagagatgatcttcgtcatcttttttatagctgtaaccttcatttctatccttacaacaggagaaggagagggcagggtgggaatcatcctcacgctggctatgaacataatgtccaccttgcagtgggccgtgaattccagtatagatgtggattctctaatgaggagtgtctcccgggtgtttaaattcattgatatgcctactgaggggaaacccaccaagtcaacaaagccttataagaatggacagctgagcaaggtgatgataattgagaacagccacgtgaagaaggatgacatttggcccagcgggggccagatgactgtgaaggacctgacggccaagtacaccgaaggtggaaatgccattttggaaaacatcagcttctcaatctctcctgggcagagagttggattgctgggtcgcacgggcagcggcaaatcaaccctgctcagtgccttccttcggctcctgaatacagaaggcgaaatccaaattgacggggtgagctgggacagcatcaccctgcagcagtggagaaaagcatttggggtcattccacagaaagttttcatcttctctggcactttcagaaagaacctggacccctatgagcagtggagcgaccaggagatctggaaggttgcagatgaagttggcctgcggagtgtgatagaacaatttcctggcaagctggattttgtgctggtagatggaggctgcgtgctgtcccacggccacaaacagctgatgtgcctcgcccgctccgttctttcaaaggccaaaatcttgcttttggatgagcccagtgctcacctcgacccagtgacctatcagataatccgcaggaccttaaagcaagcttttgccgactgcaccgtcatactgtgtgagcaccggattgaagcaatgctggaatgccagcagtttctggtgatcgaggagaataaggtccggcagtacgacagcatccagaagttgttgaatgagcgcagccttttccgccaggccatctccccatctgacagagtcaagctgtttccacataggaactcctctaagtgcaagtccaagccccagatcgctgccctcaaggaggaaactgaggaagaggtgcaggatacccgcctgtga

SEQ ID NO: 28 - DNA, 4443 bp, Synthetic Oligonucleotide
atgcagaggagcccactggagaaagcctccgtggtgagtaaactcttttttagttggaccagacccatcctgcgaaaaggatacaggcagcgcctcgagttgtcagatatctaccagattccttctgtggactcagctgacaatttgagtgagaagctggagcgggagtgggatagagagctggcgagcaaaaaaaaccccaagcttatcaatgctctgcgccgctgctttttctggaggttcatgttttatgggatcttcctgtacctgggggaggtcaccaaagctgttcagccgctccttcttggccgcatcatcgccagctatgaccctgataataaagaagaaaggtctattgctatttatctgggaattggcctctgcttgctcttcatcgtccgcacccttctgctgcaccctgccatttttggccttcaccacatcggcatgcaaatgagaattgccatgttctccctcatttacaaaaagaccctgaaactttcctcaagagtgttagataaaatatccattggtcagctggtcagcctgctgtccaacaatcttaacaaatttgatgaaggcttggcgctggcccacttcgtgtggattgcacctctgcaggtggccctgttgatgggacttatatgggagctgcttcaagcctctgctttctgtgggctgggctttttgattgtactggcactttttcaggctgggctcggaagaatgatgatgaaatacagagatcagcgggccgggaagatatcagagcgacttgtgatcaccagtgaaatgattgaaaatattcagagcgtgaaagcctactgctgggaagaagccatggagaagatgattgagaacctgaggcagacagagctcaagctcactcggaaggctgcttatgttcgctatttcaacagcagcgccttcttcttcagtggcttctttgttgtcttcctgtctgttctgccatatgcactgataaaaggcattattttacgaaagatcttcaccaccatcagtttttgcatcgttctcaggatggccgtcacaagacagttcccctgggctgtgcagacctggtacgattccttgggggccatcaacaagattcaagatttcttgcaaaaacaagaatataaaactttagaatacaacctcaccaccactgaagtggtcatggaaaatgtgacagccttttgggaggagggttttggagaattgttcgagaaggcaaagcagaataacaacaacaggaagacgagcaatggggacgactctctcttcttcagcaacttttcactgctcgggacccctgtgttgaaagatataaacttcaagatcgagaggggccagctcttggctgtggcaggctccactggagctggtaaaacatctcttctcatggtgatcatgggggaactggagccttccgaaggaaaaatcaagcacagtgggagaatctcattctgcagccagttttcctggatcatgcccggcaccattaaggaaaacatcatatttggagtgtcctatgatgagtaccgctaccggtcagtcatcaaagcctgtcagttggaggaggacatctccaagtttgcagagaaagacaacattgtgcttggagaggggggtatcactctttctggaggacaaagagccaggatctctttggcccgggcagtctacaaggatgcagacctctacttgttggacagtcccttcggctacctcgacgtgctgactgaaaaagaaatttttgaaagctgtgtgtgcaaactgatggcaaacaagaccaggattcttgtcaccagcaagatggaacatctgaagaaagcggacaaaattctgattctgcatgaagggagctcctacttctatggaacatttagcgagcttcagaacctacagccagacttctcctccaaattaatgggctgtgactccttcgaccagttctctgcagaaagaagaaactctatactcacagagaccctccaccgcttctcccttgagggagatgccccagtttcttggacagaaaccaagaagcagtcctttaagcagactggcgagtttggtgaaaagaggaaaaattcaattctcaatcctattaacagtattcgcaagttcagcattgtccagaagacacccctccagatgaatggcatcgaagaagatagtgacgagccgctggagagacggctgagtctggtgccagattcagaacagggggaggccatcctgccccggatcagcgtcatttccacaggccccacattacaagcacggcgccggcagagtgttttaaatctcatgacccattcagtgaaccagggccaaaatatccacaggaagactacagcttctacccggaaagtgtctctggcccctcaggccaatctgaccgagctggacatctacagcaggaggctctcccaggaaacagggcttgaaatatctgaagagattaatgaagaggatcttaaagagtgcttctttgatgacatggagagcatccccgcggtgaccacatggaacacctaccttagatatattactgtccacaagagcctcatatttgtcctcatctggtgcctggttattttcctcgctgaggtggcggccagtcttgttgtgctctggctgctgggcaacactcctctccaggacaagggcaatagtacacacagcagaaataattcttatgccgtcatcattacaagcacctccagctactacgtgttctacatctatgtgggcgtggctgacaccctcctggccatgggtttcttccggggcctgcctttggtgcacaccctcatcacagtgtcaaaaattctgcaccataaaatgcttcattctgtcctgcaggcacccatgagcactttgaacacattgaaggctggcggcatcctcaacagattttctaaagatattgctatcctggatgatctcctccccctgacaatctttgactttatccagcttctgctgatcgtgattggagccatagcagtggttgctgtcctgcagccctacatttttgtggccaccgtgcccgtgattgttgcctttattatgctcagagcttacttcctgcaaacttctcaacagctcaaacagctagaatctgagggccggagccccatttttacccacctggtgacttccctgaagggactgtggactctgagagcattcgggcgacagccttactttgagacactgttccacaaggccctgaacttgcacactgccaactggtttctttacctgagcacactccgctggttccagatgcggatagagatgatcttcgtcatcttttttatagctgtaaccttcatttctatccttacaacaggagaaggagagggcagggtgggaatcatcctcacgctggctatgaacataatgtccaccttgcagtgggccgtgaattccagtatagatgtggattctctaatgaggagtgtctcccgggtgtttaaattcattgatatgcctactgaggggaaacccaccaagtcaacaaaaccttataagaatggacagctgagcaaggtgatgataattgagaacagccacgtgaagaaggatgacatttggcccagcgggggccagatgactgtgaaggacctgacggccaagtacaccgaaggtggaaatgccattttggaaaacatcagcttctcaatctctcctgggcagagagttggattgctgggtcgcacgggcagcggcaaatcaaccctgctcagtgccttccttcggctcctgaatacagaaggcgaaatccaaattgacggggtgagctgggacagcatcaccctgcagcagtggagaaaagcatttggggtcattccacagaaagttttcatcttctctggcactttcagaaagaacctggacccctatgagcagtggagcgaccaggagatctggaaggttgcagatgaagttggcctgcggagtgtgatagaacaatttcctggcaagctggattttgtgctggtagatggaggctgcgtgctgtcccacggccacaaacagctgatgtgcctcgcccgctccgttctttcaaaggccaaaatcttgcttttggatgagcccagtgctcacctcgacccagtgacctatcagataatccgcaggaccttaaagcaagcttttgccgactgcaccgtcatactgtgtgagcaccggattgaagcaatgctggaatgccagcagtttctggtgatcgaggagaataaggtccggcagtacgacagcatccagaagttgttgaatgagcgcagccttttccgccaggccatctccccatctgacagagtcaagctgtttccacataggaactcctctaagtgcaagtccaagccccagatcgctgccctcaaggaggaaactgaggaagaggtgcaggatacccgcctgtga

SEQ ID NO: 29 - DNA, 4443 bp, Synthetic Oligonucleotide
atgcagaggagcccactggagaaagcctccgtggtgagtaaactcttttttagttggaccagacccatcctgcgaaaaggatacaggcagcgcctcgagttgtcagatatctaccagattccttctgtggactcagctgacaatttgagtgagaagctggagcgggagtgggatagagagctggcgagcaaaaaaaaccccaagcttatcaatgctctgcgccgctgctttttctggaggttcatgttttatgggatcttcctgtacctgggggaggtcaccaaagctgttcagccgctccttcttggccgcatcatcgccagctatgaccctgataataaagaagaaaggtctattgctatttatctgggaattggcctctgcttgctcttcatcgtccgcacccttctgctgcaccctgccatttttggccttcaccacatcggcatgcaaatgagaattgccatgttctccctcatttacaaaaagaccctgaaactttcctcaagagtgttagataaaatatccattggtcagctggtcagcctgctgtccaacaatcttaacaaatttgatgaaggcttggcgctggcccacttcgtgtggattgcacctctgcaggtggccctgttgatgggacttatatgggagctgcttcaagcctctgctttctgtgggctgggctttttgattgtactggcactttttcaggctgggctcggaagaatgatgatgaaatacagagatcagcgggccgggaagatatcagagcgacttgtgatcaccagtgaaatgattgaaaatattcagagcgtgaaagcctactgctgggaagaagccatggagaagatgattgagaacctgaggcagacagagctcaagctcactcggaaggctgcttatgttcgctatttcaacagcagcgccttcttcttcagtggcttctttgttgtcttcctgtctgttctgccatatgcactgataaaaggcattattttacgaaagatcttcaccaccatcagtttttgcatcgttctcaggatggccgtcacaagacagttcccctgggctgtgcagacctggtacgattccttgggggccatcaacaagattcaagatttcttgcaaaaacaagaatataaaactttagaatacaacctcaccaccactgaagtggtcatggaaaatgtgacagccttttgggaggagggttttggagaattgttcgagaaggcaaagcagaataacaacaacaggaagacgagcaatggggacgactctctcttcttcagcaacttttcactgctcgggacccctgtgttgaaagatataaacttcaagatcgagaggggccagctcttggctgtggcaggctccactggagctggtaaaacatctcttctcatggtgatcatgggggaactggagccttccgaaggaaaaatcaagcacagtgggagaatctcattctgcagccagttttcctggatcatgcccggcaccattaaggaaaacatcatatttggagtgtcctatgatgagtaccgctaccggtccgtcatcaaagcctgtcagttggaggaggacatctccaagtttgcagagaaagacaacattgtgcttggagaggggggtatcactctttctggaggacaaagagccaggatctctttggcccgggcagtctacaaggatgcagacctctacttgttggacagtcccttcggctacctcgacgtgctgactgaaaaagaaatttttgaaagctgtgtgtgcaaactgatggcaaacaagaccaggattcttgtcaccagcaagatggaacatctgaagaaagcggacaaaattctgattctgcatgaagggagctcctacttctatggaacatttagcgagcttcagaacctacagccagacttctcctccaaattaatgggctgtgactccttcgaccagttctctgcagaaagaagaaactctatactcacagagaccctccaccgcttctcccttgagggagatgccccagtttcttggacagaaaccaagaagcagtcctttaagcagactggcgagtttggtgaaaagaggaaaaattcaattctcaatccaattaacagtattcgcaagttcagcattgtccagaagacacccctccagatgaatggcatcgaagaagatagtgacgagccgctggagagacggctgagtctggtgccagattcagaacagggggaggccatcctgccccggatcagcgtcatttccacaggccccacattacaagcacggcgccggcagagtgttttaaatctcatgacccattcagtgaaccagggccaaaatatccacaggaagactacagcttctacccggaaagtgtctctggcccctcaggccaatctgaccgagctggacatctacagcaggaggctctcccaggaaacagggctggaaatatctgaagagattaatgaagaggatcttaaagagtgcttctttgatgacatggagagcatccccgcggtgaccacatggaacacctaccttagatatattactgtccacaagagcctcatatttgtcctcatctggtgcctggttattttcctcgctgaggtggcggccagtcttgttgtgctctggctgctgggcaacactcctctccaggacaagggcaatagtactcacagcagaaataattcttatgccgtcatcattacaagcacctccagctactacgtgttctacatctatgtgggcgtggctgacaccctcctggccatgggtttcttccggggcctgcctttggtgcacaccctcatcacagtgtcaaaaattctgcaccataaaatgcttcattctgtcctgcaggcacccatgagcactttgaacacattgaaggctggcggcatcctcaacagattttctaaagatattgctatcctggatgatctcctccccctgacaatctttgactttatccagcttctgctgatcgtgattggagccatagcagtggttgctgtcctgcagccctacatttttgtggccaccgtgcccgtgattgttgcctttattatgctcagagcttacttcctgcaaacttctcaacagctcaaacagctagagtctgagggccggagccccatttttacccacctggtgacttccctgaagggactgtggactctgagagcattcgggcgacagccttactttgagacactgttccacaaggccctgaacttgcacactgccaactggtttctttacctgagcacactccgctggttccagatgcggatagagatgatcttcgtcatcttttttatagctgtaaccttcatttctatccttacaacaggagaaggagagggcagggtgggaatcatcctcacgctggctatgaacataatgtccaccttgcagtgggccgtgaattccagtatagatgtggattctctaatgaggagtgtctcccgggtgtttaaattcattgatatgcctactgaggggaaacccaccaagtcaacaaaaccttataagaatggacagctgagcaaggtgatgataattgagaacagccacgtgaagaaggatgacatttggcccagcgggggccagatgactgtgaaggacctgacggccaagtacaccgaaggtggaaatgccattttggaaaacatcagcttctcaatctctcctgggcagagagttggattgctgggtcgcacgggcagcggcaaatcaaccctgctcagtgccttccttcggctcctgaatacagaaggcgaaatccaaattgacggggtgagctgggacagcatcaccctgcagcagtggagaaaagcatttggggtcattccacagaaagttttcatcttctctggcactttcagaaagaacctggacccctatgagcagtggagcgaccaggagatctggaaggttgcagatgaagttggcctgcggagtgtgatagaacaatttcctggcaagctggattttgtgctggtagatggaggctgcgtgctgtcccacggccacaaacagctgatgtgcctcgcccgctccgttctttcaaaggccaaaatcttgcttttggatgagcccagtgctcacctcgacccagtgacctatcagataatccgcaggaccttaaagcaagcttttgccgactgcaccgtcatactgtgtgagcaccggattgaagcaatgctggaatgccagcagtttctggtgatcgaggagaataaggtccggcagtacgacagcatccagaagttgttgaatgagcgcagccttttccgccaggccatctccccatctgacagagtcaagctgtttccacataggaactcctctaagtgcaagtccaagccccagatcgctgccctcaaggaggaaactgaggaagaggtgcaggatacccgcctgtga

SEQ ID NO: 30 - DNA, 4443 bp, Synthetic Oligonucleotide
atgcagaggagcccactggagaaagcctccgtggtgagtaaactcttttttagttggaccagacccatcctgcgaaaaggatacaggcagcgcctcgagttgtctgatatctaccagattccttctgtggactcagctgacaatttgagtgagaagctggagcgggagtgggatagagagctggcgagcaaaaaaaaccccaagcttatcaatgctctgcgccgctgctttttctggaggttcatgttttatgggatcttcctgtacctgggggaggtcaccaaagctgttcagccgctccttcttggccgcatcatcgccagctatgaccctgataataaagaagaaaggtctattgctatttatctgggaattggcctctgcttgctcttcatcgtccgcacccttctgctgcaccctgccatttttggccttcaccacatcggcatgcaaatgagaattgccatgttctccctcatttacaaaaagaccctgaaactttcctcaagagtgttagataaaatatccattggtcagctggtcagcctgctgtccaacaatcttaacaaatttgatgaaggcttggcgctggcccacttcgtgtggattgcacctctgcaggtggccctgttgatgggacttatatgggagctgcttcaagcctctgctttctgtgggctgggctttttgattgtactggcactttttcaggctgggctcggaagaatgatgatgaaatacagagatcagcgggccgggaagatttcagagcgacttgtgatcaccagtgaaatgattgaaaatattcagagcgtgaaagcctactgctgggaagaagccatggagaagatgattgagaacctgaggcagacagagctcaagctcactcggaaggctgcttatgttcgctatttcaacagcagcgccttcttcttcagtggcttctttgttgtcttcctgtctgttctgccatatgcactgataaaaggcattattttacgaaagatcttcaccaccatcagtttttgcatcgttctcaggatggccgtcacaagacagttcccctgggctgtgcagacctggtacgattccttgggggccatcaacaagattcaagatttcttgcaaaaacaagaatataaaactttagaatacaacctcaccaccactgaagtggtcatggaaaatgtgacagccttttgggaggagggttttggagaattgttcgagaaggcaaagcagaataacaacaacaggaagacgagcaatggggacgactctctcttcttcagcaacttttcactgctcgggacccctgtgttgaaagatataaacttcaagatcgagaggggccagctcttggctgtggcaggctccactggagctggtaaaacatctcttctcatggtgatcatgggggaactggagccttccgaaggaaaaatcaagcacagtgggagaatctcattctgcagccagttttcctggatcatgcccggcaccattaaggaaaacatcatatttggagtgtcctatgatgagtaccgctaccggtcagtcatcaaagcctgtcagttggaggaggacatctccaagtttgcagagaaagacaacattgtgcttggagaggggggtatcactctttctggaggacaaagagccaggatctctttggcccgggcagtctacaaggatgcagacctctacttgttggacagtcccttcggctacctcgacgtgctgactgaaaaagaaatttttgaaagctgtgtgtgcaaactgatggcaaacaagaccaggattcttgtcaccagcaagatggaacatctgaagaaagcggacaaaattctgattctgcatgaagggagctcctacttctatggaacatttagcgagcttcagaacctacagccagacttctcctccaaattaatgggctgtgactccttcgaccagttctctgcagaaagaagaaactctatactcacagagaccctccaccgcttctcccttgagggagatgccccagtttcttggacagaaaccaagaagcagtcctttaagcagactggcgagtttggtgaaaagaggaaaaattcaattctcaatcctattaacagtattcgcaagttcagcattgtccagaagacacccctccagatgaatggcatcgaagaagatagtgacgagccgctggagagacggctgagtctggtgccagattcagaacagggggaggccatcctgccccggatcagcgtcatttccacaggccccacattacaagcacggcgccggcagagtgttttaaatctcatgacccattcagtgaaccagggccaaaatatccacaggaagactacagcttctacccggaaagtgtctctggcccctcaggccaatctgaccgagctggacatctacagcaggaggctctcccaggaaacagggctggaaatatctgaagagattaatgaagaggatcttaaagagtgcttctttgatgacatggagagcatccccgcggtgaccacatggaacacctaccttagatatattactgtccacaagagcctcatatttgtcctcatctggtgcctggttattttcctcgctgaggtggcggccagtcttgttgtgctctggctgctgggcaacactcctctccaggacaagggcaatagtacacacagcagaaataattcttatgccgtcatcattacaagcacctccagctactacgtgttctacatctatgtgggcgtggctgacaccctcctggccatgggtttcttccggggcctgcctttggtgcacaccctcatcacagtgtcaaaaattctgcaccataaaatgcttcattctgtcctgcaggcacccatgagcactttgaacacattgaaggctggcggcatcctcaacagattttctaaagatattgctatcctggatgatctcctccccctgacaatctttgactttatccagcttctgctgatcgtgattggagccatagcagtggttgctgtcctgcagccctacatttttgtggccaccgtgcccgtgattgttgcctttattatgctcagagcttacttcctgcaaacttctcaacagctcaaacagctagaatctgagggccggagccccatttttacccacctggtgacttccctgaagggactgtggactctgagagcattcgggcgacagccttactttgagacactgttccacaaggccctgaacttgcacactgccaactggtttctttacctgagcacactccgctggttccagatgcggatagagatgatcttcgtcatcttttttatagctgtaaccttcatttctatccttacaacaggagaaggagagggcagggtgggaatcatcctcacgctggctatgaacataatgtccaccttgcagtgggccgtgaattccagtatagatgtggattctctaatgaggagtgtctcccgggtgtttaaattcattgatatgcctactgaggggaaacccaccaagtcaacaaaaccttataagaatggacagctgagcaaggtgatgataattgagaacagccacgtgaagaaggatgacatttggcccagcgggggccagatgactgtgaaggacctgacggccaagtacaccgaaggtggaaatgccattttggaaaacatcagcttctcaatctctcctgggcagagagttggattgctgggtcgcacgggcagcggcaaatcaaccctgctcagtgccttccttcggctcctgaatacagaaggcgaaatccaaattgacggggtgagctgggacagcatcaccctgcagcagtggagaaaagcatttggggtcattccacagaaagttttcatcttctctggcactttcagaaagaacctggacccctatgagcagtggagcgaccaggagatctggaaggttgcagatgaagttggcctgcggagtgtgatagaacaatttcctggcaagctggattttgtgctggtagatggaggctgcgtgctgtcccacggccacaaacagctgatgtgcctcgcccgctccgttctttcaaaggccaaaatcttgcttttggatgagcccagtgctcacctcgacccagtgacctatcagataatccgcaggaccttaaagcaagcttttgccgactgcaccgtcatactgtgtgagcaccggattgaagcaatgctggaatgccagcagtttctggtgatcgaggagaataaggtccggcagtacgacagcatccagaagttgttgaatgagcgcagccttttccgccaggccatctccccatctgacagagtcaagctgtttccacataggaactcctctaagtgcaagtccaagccccagatcgctgccctcaaggaggaaactgaggaagaggtgcaggatacccgcctgtga

SEQ ID NO: 31 - DNA, 4443 bp, Synthetic Oligonucleotide
atgcagagaagccccctggagaaggcctctgtggtgagcaagctgttcttcagctggaccagacccatcctgagaaagggctacagacagagactggagctgtctgacatctaccagatcccctctgtggactctgccgacaacctgtctgagaagctggagagagagtgggacagagagctggccagcaagaagaaccccaagctgatcaatgccctgagaagatgcttcttctggagattcatgttctatggcatcttcctgtacctgggagaggtgaccaaggccgtgcagcccctgctgctgggcaggatcattgccagctatgaccctgacaacaaggaggagagaagcattgccatctacctgggcattggcctgtgcctgctgttcattgtgagaaccctgctgctgcaccctgccatctttggcctgcaccacattggcatgcagatgagaattgccatgttcagcctgatctacaagaagaccctgaagctgagcagcagagtgctggacaagatcagcattggccagctggtgagcctgctgagcaacaacctgaacaagtttgatgagggcctggccctggcccactttgtgtggattgcccccctgcaggtggccctgctgatgggcctgatctgggagctgctgcaggcctctgccttctgtggcctgggcttcctgattgtgctggccctgttccaggccggcctgggcagaatgatgatgaagtacagagaccagagagccggcaagatctctgagagactggtgatcacctctgagatgattgagaacatccagtctgtgaaggcctactgctgggaggaggccatggagaagatgattgagaacctgagacagacagagctgaagctgaccaggaaggccgcctatgtgagatacttcaacagctctgccttcttcttctctggcttctttgtggtgttcctgtctgtgctgccctatgccctgatcaagggcatcatcctgaggaagatcttcaccaccatcagcttctgcattgtgctgaggatggccgtgaccaggcagttcccctgggccgtgcagacctggtatgacagcctgggggccatcaacaagatccaggacttcctgcagaagcaggagtacaagaccctggagtacaacctgaccaccacagaggtggtgatggagaatgtgacagccttctgggaggagggctttggagagctgtttgagaaggccaagcagaacaacaacaacagaaagaccagcaatggagatgacagcctgttcttcagcaacttcagcctgctgggcacccctgtgctgaaggacatcaacttcaagattgagaggggccagctgctggccgtggccggcagcacaggagccggcaagaccagcctgctgatggtgatcatgggagagctggagccctctgagggcaagatcaagcactctggcagaatcagcttctgcagccagttcagctggatcatgcctggcaccatcaaggagaacatcatctttggggtgagctatgatgagtacaggtacagatctgtgatcaaggcctgccagctggaggaggacatctccaagtttgccgagaaggacaacattgtgctgggggagggaggcatcaccctgtctgggggccagagagccagaatcagcctggccagagccgtgtacaaggatgccgacctgtacctgctggacagcccctttggctacctggatgtgctgacagagaaggagatctttgagagctgtgtgtgcaagctgatggccaacaagaccaggatcctggtgaccagcaagatggagcacctgaagaaggccgacaagatcctgatcctgcatgagggcagcagctacttctatggcaccttctctgagctgcagaacctgcagcctgacttcagcagcaagctgatgggctgtgacagctttgaccagttctctgctgagagaagaaacagcatcctgacagagaccctgcacaggttcagcctggagggggatgcccctgtgagctggacagagaccaagaagcagagcttcaagcagacaggagagtttggggagaagaggaagaacagcatcctgaaccccatcaacagcatcaggaagttcagcattgtgcagaagacccccctgcagatgaatggcattgaggaggactctgatgagcccctggagagaagactgagcctggtgccagactctgagcagggagaggccatcctgcccaggatctctgtgatcagcacaggccccaccctgcaggccagaagaagacagtctgtgctgaacctgatgacccactctgtgaaccagggccagaatatccacagaaagaccacagccagcaccagaaaggtgagcctggccccccaggccaacctgacagagctggacatctacagcagaaggctgagccaggagacaggcctggagatctctgaggagatcaatgaggaggacctgaaggagtgcttctttgatgacatggagagcatccctgccgtgaccacctggaacacctacctgagatacatcacagtgcacaagagcctgatctttgtgctgatctggtgcctggtgatcttcctggccgaggtggccgccagcctggtggtgctgtggctgctgggcaacacccccctgcaggacaagggcaacagcacccacagcagaaacaacagctatgctgtgatcatcaccagcaccagcagctactatgtgttctacatctatgtgggagtggctgacaccctgctggccatgggcttcttcagaggcctgcccctggtgcacaccctgatcacagtgagcaagatcctgcaccacaagatgctgcactctgtgctgcaggcccccatgagcaccctgaacaccctgaaggctggaggcatcctgaacagattcagcaaggacattgccatcctggatgacctgctgcccctgaccatctttgacttcatccagctgctgctgattgtgattggagccattgccgtggtggccgtgctgcagccctacatctttgtggccacagtgcctgtgattgtggccttcatcatgctgagggcctacttcctgcagaccagccagcagctgaagcagctggagtctgagggcagaagccccatcttcacccacctggtgaccagcctgaagggcctgtggaccctgagggcctttggcagacagccctactttgagaccctgttccacaaggccctgaacctgcacacagccaactggttcctgtacctgagcaccctgagatggttccagatgaggattgagatgatctttgtgatcttcttcattgccgtgaccttcatcagcatcctgaccacaggggagggcgagggcagagtgggcatcatcctgaccctggccatgaacatcatgagcaccctgcagtgggccgtgaacagcagcattgatgtggacagcctgatgagatctgtgagcagagtgttcaagttcattgacatgcccacagagggcaagcccaccaagagcaccaagccctacaagaatggccagctgagcaaggtgatgatcattgagaacagccatgtgaagaaggatgacatctggccctctggaggccagatgacagtgaaggacctgacagccaagtacacagaggggggcaatgccatcctggagaacatcagcttcagcatcagccctggccagagggtgggcctgctgggcagaacaggctctggcaagagcaccctgctgtctgccttcctgaggctgctgaacacagagggagagatccagattgatggggtgagctgggacagcatcaccctgcagcagtggaggaaggcctttggggtgatcccccagaaggtgttcatcttctctggcaccttcaggaagaacctggacccctatgagcagtggtctgaccaggagatctggaaggtggccgatgaggtgggcctgagatctgtgattgagcagttccctggcaagctggactttgtgctggtggatggaggctgtgtgctgagccatggccacaagcagctgatgtgcctggccagatctgtgctgagcaaggccaagatcctgctgctggatgagccctctgcccacctggaccctgtgacctaccagatcatcagaagaaccctgaagcaggcctttgccgactgcacagtgatcctgtgtgagcacagaattgaggccatgctggagtgccagcagttcctggtgattgaggagaacaaggtgaggcagtatgacagcatccagaagctgctgaatgagagaagcctgttcagacaggccatcagcccctctgacagagtgaagctgttcccccacaggaacagcagcaagtgcaagagcaagccccagattgccgccctgaaggaggagacagaggaggaggtgcaggacaccagactgtga

SEQ ID NO: 32 - DNA, 4443 bp, Synthetic Oligonucleotide
atgcagaggagccccctggagaaggccagcgtggtgagcaagctgttcttcagctggaccaggcccatcctgaggaagggctacaggcagaggctggagctgagcgacatctaccagatccccagcgtggacagcgccgacaacctgagcgagaagctggagagggagtgggacagggagctggccagcaagaagaaccccaagctgatcaacgccctgaggaggtgcttcttctggaggttcatgttctacggcatcttcctgtacctgggcgaggtgaccaaggccgtgcagcccctgctgctgggcaggatcatcgccagctacgaccccgacaacaaggaggagaggagcatcgccatctacctgggcatcggcctgtgcctgctgttcatcgtgaggaccctgctgctgcaccccgccatcttcggcctgcaccacatcggcatgcagatgaggatcgccatgttcagcctgatctacaagaagaccctgaagctgagcagcagggtgctggacaagatcagcatcggccagctggtgagcctgctgagcaacaacctgaacaagttcgacgagggcctggccctggcccacttcgtgtggatcgcccccctgcaggtggccctgctgatgggcctgatctgggagctgctgcaggccagcgccttctgcggcctgggcttcctgatcgtgctggccctgttccaggccggcctgggcaggatgatgatgaagtacagggaccagagggccggcaagatcagcgagaggctggtgatcaccagcgagatgatcgagaacatccagagcgtgaaggcctactgctgggaggaggccatggagaagatgatcgagaacctgaggcagaccgagctgaagctgaccaggaaggccgcctacgtgaggtacttcaacagcagcgccttcttcttcagcggcttcttcgtggtgttcctgagcgtgctgccctacgccctgatcaagggcatcatcctgaggaagatcttcaccaccatcagcttctgcatcgtgctgaggatggccgtgaccaggcagttcccctgggccgtgcagacctggtacgacagcctgggcgccatcaacaagatccaggacttcctgcagaagcaggagtacaagaccctggagtacaacctgaccaccaccgaggtggtgatggagaacgtgaccgccttctgggaggagggcttcggcgagctgttcgagaaggccaagcagaacaacaacaacaggaagaccagcaacggcgacgacagcctgttcttcagcaacttcagcctgctgggcacccccgtgctgaaggacatcaacttcaagatcgagaggggccagctgctggccgtggccggcagcaccggcgccggcaagaccagcctgctgatggtgatcatgggcgagctggagcccagcgagggcaagatcaagcacagcggcaggatcagcttctgcagccagttcagctggatcatgcccggcaccatcaaggagaacatcatcttcggcgtgagctacgacgagtacaggtacaggagcgtgatcaaggcctgccagctggaggaggacatcagcaagttcgccgagaaggacaacatcgtgctgggcgagggcggcatcaccctgagcggcggccagagggccaggatcagcctggccagggccgtgtacaaggacgccgacctgtacctgctggacagccccttcggctacctggacgtgctgaccgagaaggagatcttcgagagctgcgtgtgcaagctgatggccaacaagaccaggatcctggtgaccagcaagatggagcacctgaagaaggccgacaagatcctgatcctgcacgagggcagcagctacttctacggcaccttcagcgagctgcagaacctgcagcccgacttcagcagcaagctgatgggctgcgacagcttcgaccagttcagcgccgagaggaggaacagcatcctgaccgagaccctgcacaggttcagcctggagggcgacgcccccgtgagctggaccgagaccaagaagcagagcttcaagcagaccggcgagttcggcgagaagaggaagaacagcatcctgaaccccatcaacagcatcaggaagttcagcatcgtgcagaagacccccctgcagatgaacggcatcgaggaggacagcgacgagcccctggagaggaggctgagcctggtgcccgacagcgagcagggcgaggccatcctgcccaggatcagcgtgatcagcaccggccccaccctgcaggccaggaggaggcagagcgtgctgaacctgatgacccacagcgtgaaccagggccagaacatccacaggaagaccaccgccagcaccaggaaggtgagcctggccccccaggccaacctgaccgagctggacatctacagcaggaggctgagccaggagaccggcctggagatcagcgaggagatcaacgaggaggacctgaaggagtgcttcttcgacgacatggagagcatccccgccgtgaccacctggaacacctacctgaggtacatcaccgtgcacaagagcctgatcttcgtgctgatctggtgcctggtgatcttcctggccgaggtggccgccagcctggtggtgctgtggctgctgggcaacacccccctgcaggacaagggcaacagcacccacagcaggaacaacagctacgccgtgatcatcaccagcaccagcagctactacgtgttctacatctacgtgggcgtggccgacaccctgctggccatgggcttcttcaggggcctgcccctggtgcacaccctgatcaccgtgagcaagatcctgcaccacaagatgctgcacagcgtgctgcaggcccccatgagcaccctgaacaccctgaaggccggcggcatcctgaacaggttcagcaaggacatcgccatcctggacgacctgctgcccctgaccatcttcgacttcatccagctgctgctgatcgtgatcggcgccatcgccgtggtggccgtgctgcagccctacatcttcgtggccaccgtgcccgtgatcgtggccttcatcatgctgagggcctacttcctgcagaccagccagcagctgaagcagctggagagcgagggcaggagccccatcttcacccacctggtgaccagcctgaagggcctgtggaccctgagggccttcggcaggcagccctacttcgagaccctgttccacaaggccctgaacctgcacaccgccaactggttcctgtacctgagcaccctgaggtggttccagatgaggatcgagatgatcttcgtgatcttcttcatcgccgtgaccttcatcagcatcctgaccaccggcgagggcgagggcagggtgggcatcatcctgaccctggccatgaacatcatgagcaccctgcagtgggccgtgaacagcagcatcgacgtggacagcctgatgaggagcgtgagcagggtgttcaagttcatcgacatgcccaccgagggcaagcccaccaagagcaccaagccctacaagaacggccagctgagcaaggtgatgatcatcgagaacagccacgtgaagaaggacgacatctggcccagcggcggccagatgaccgtgaaggacctgaccgccaagtacaccgagggcggcaacgccatcctggagaacatcagcttcagcatcagccccggccagagggtgggcctgctgggcaggaccggcagcggcaagagcaccctgctgagcgccttcctgaggctgctgaacaccgagggcgagatccagatcgacggcgtgagctgggacagcatcaccctgcagcagtggaggaaggccttcggcgtgatcccccagaaggtgttcatcttcagcggcaccttcaggaagaacctggacccctacgagcagtggagcgaccaggagatctggaaggtggccgacgaggtgggcctgaggagcgtgatcgagcagttccccggcaagctggacttcgtgctggtggacggcggctgcgtgctgagccacggccacaagcagctgatgtgcctggccaggagcgtgctgagcaaggccaagatcctgctgctggacgagcccagcgcccacctggaccccgtgacctaccagatcatcaggaggaccctgaagcaggccttcgccgactgcaccgtgatcctgtgcgagcacaggatcgaggccatgctggagtgccagcagttcctggtgatcgaggagaacaaggtgaggcagtacgacagcatccagaagctgctgaacgagaggagcctgttcaggcaggccatcagccccagcgacagggtgaagctgttcccccacaggaacagcagcaagtgcaagagcaagccccagatcgccgccctgaaggaggagaccgaggaggaggtgcaggacaccaggctgtga

SEQ ID NO: 33 - DNA, 4443 bp, Synthetic Oligonucleotide
atgcagagatcccctctggagaaggcctcagtggtgtccaagcttttcttctcctggaccaggcccattttaagaaagggctacaggcagagacttgagctgtctgacatctatcagatcccttctgtggattctgctgacaatcttagtgaaaaattggaaagggagtgggacagagagctggcaagtaaaaagaaccccaagctgattaatgccctgaggcgctgctttttttggagattcatgttctatggcatattcctctaccttggagaagtaaccaaagctgtacagcctctcctccttggcagaatcattgcctcctatgatcctgataacaaggaggagagaagcatagccatctacctgggcattgggctgtgcctcttgtttattgtgaggacccttctcttgcaccctgccatctttggccttcatcacattggcatgcaaatgagaatagcaatgtttagtcttatttacaaaaaaacattaaaactctcttccagggtgttggacaagatcagtattggacaactggtcagcctgctgagcaacaacctgaacaagtttgatgaaggactggccctggcccactttgtctggattgccccccttcaggtggctcttttgatgggcctgatctgggaactcctgcaggcctctgccttctgtgggttaggcttcctgatagtgctagctctctttcaggcagggttgggtagaatgatgatgaagtacagagaccagagggctgggaagatatctgagaggctggtcattacttctgaaatgatagaaaacatccagtctgttaaagcttactgctgggaggaggctatggaaaagatgattgagaacttgaggcaaacagagctcaagctgactaggaaggcagcctatgtcaggtatttcaacagcagtgctttcttcttctcaggctttttcgtggtcttcttgagtgttctgccctatgccctcatcaaggggataattttgagaaagattttcaccactatttccttttgcattgtcctgaggatggctgtcaccaggcaattcccctgggctgtgcagacatggtatgactctctgggggccatcaacaaaatccaagatttcctgcagaagcaggagtacaagaccctggaatacaacctcaccaccacagaagttgtgatggagaatgtgactgcattctgggaggaaggatttggggagctgtttgagaaagcaaaacaaaacaataataacaggaaaaccagcaatggagatgactccctgttcttttccaacttctctttgttgggcacccctgtcctgaaagatataaactttaaaattgaaagagggcagctgttggcagttgctggctccacaggagctggaaaaacttcactactgatggtgatcatgggggagttagaaccctctgaagggaaaataaaacattctgggaggattagtttctgcagccagttcagctggatcatgcctgggaccattaaagaaaatattatatttggagtgagctatgatgaatatagatataggagtgtcatcaaagcctgtcagttggaggaagacatcagcaaatttgcagagaaagacaacattgttctgggtgaaggtggcatcaccctgtcaggagggcaaagggccaggatcagcttggccagagcagtctataaagatgctgatctgtacctcctggatagcccttttggctatctggatgttttgacagagaaggaaatttttgagtcctgtgtctgcaagttaatggcaaataaaacaaggatacttgtgacctcaaaaatggaacacctgaagaaggctgacaaaattctgatcctgcatgagggcagcagctacttttatggaacattttctgaactgcagaatttgcaaccagacttttcatcaaagctcatgggatgtgacagttttgatcagttttctgcagaaaggagaaactccattttgactgagaccctgcacaggttcagtctggagggggatgccccagtgagttggactgagacaaagaaacagagcttcaagcagactggagagtttggagaaaagaggaaaaactcaattctcaatcccatcaatagcatcaggaagttcagcatagttcagaagactcctttgcagatgaatgggattgaagaggactcagatgagcccctggaaaggagactctccttggtgccagattcagagcagggggaagccatactgccaaggatctctgtgatttctacagggcccaccctccaagcaagaaggagacagtcagttttaaacctgatgacccactctgtcaaccagggacagaacattcatagaaagacaacagcatctacaagaaaagtttcactggcccctcaagccaatttaactgaactagatatctacagcaggaggctcagccaagaaacaggcctggagatctcagaagaaataaatgaggaggatttgaaggaatgcttctttgatgatatggagagcatcccagctgtcacaacctggaacacctacctgagatacatcacagtgcacaaatccctcatctttgtacttatatggtgccttgtcatcttcttagctgaggtggctgcttccctggtggtgctgtggctgctgggaaacacacccctccaggataaagggaactctactcacagcaggaacaacagttatgctgtgatcatcaccagtacctcctcctactatgtgttctacatttatgttggagttgcagacacattgcttgccatgggtttttttagaggactccccctggtgcatactctcatcactgtttccaaaatccttcaccacaagatgctgcacagtgtactacaggctcccatgagcaccctcaacactcttaaagcaggaggaatcttgaacagatttagcaaggacattgcaattcttgatgacctgcttccactgaccatctttgacttcatccagcttctgctcattgtaattggtgccattgctgtggtagcagtgctccagccatatatttttgtggccactgtgcctgttattgtggccttcattatgttgagagcctacttcctgcagacctctcagcagctcaagcaacttgaaagtgagggcaggagccccatatttacacacttggtcacttccctcaaaggcctctggacactcagagcttttggaagacaaccttattttgaaactctcttccacaaggctctgaatctccacacagccaactggtttctgtatctttcaacactgcgctggttccagatgaggattgagatgatctttgttatcttcttcatagctgttaccttcatctctattctgacaactggtgagggggaagggagagtaggcatcatcctcacactagccatgaacataatgtctaccttacaatgggccgtgaacagctccatagatgtggacagcctcatgagaagtgtgtcaagagttttcaaattcattgacatgcccacagaaggcaaaccaaccaagagcacaaaaccctacaagaatggccagctgagtaaggtcatgatcattgaaaattctcatgtgaagaaggatgatatttggcccagtgggggccagatgacagtcaaggacctcactgccaaatacacagagggtggaaatgctatcctagagaacatctccttctccatctccccaggccaaagagttggcttgctgggcaggactggcagtggcaagtccaccttgctctcagcatttctcaggcttttaaatacagagggagagattcaaattgatggggtgtcttgggatagtataacacttcaacagtggaggaaagcctttggtgtgattcctcagaaagtgtttatcttctctggcactttcagaaaaaatctggacccctatgaacagtggagtgaccaggaaatctggaaggtggcagatgaagtgggcctaagatcagtcatagagcagtttcctggaaagttggattttgtgcttgtagatggaggctgtgtgctgtcccatggccataaacagctaatgtgcctggctaggtcagtgctgagcaaggccaagatcctgctgttagatgagccttcagcccatctggaccctgtgacataccagattatcagaagaactctgaagcaggcctttgctgactgcactgtcatcctgtgtgagcacagaattgaggccatgctggagtgccagcagttccttgttatagaagagaataaggttaggcagtatgacagcattcagaaactgctaaatgaaagatctctcttcaggcaagctatttcaccatctgatagagtgaaactttttccccacagaaattcctctaaatgtaaatctaagccccagatagctgccttgaaagaggagactgaagaagaagtccaggacaccagactgtga

SEQ ID NO: 34 - DNA, 4443 bp, Synthetic Oligonucleotide
atgcagagatccccgctggagaaggcatctgtggtgtcaaaactgttctttagctggacaaggcccatccttaggaaagggtacagacagaggttggagctgtcagacatatatcagatcccttcagtggactctgcagacaacctctctgaaaagctggagagggaatgggacagggaactggccagcaaaaaaaaccctaaactgattaatgccctgaggaggtgcttcttttggagattcatgttctatgggatcttcctttacctgggggaggtgactaaagctgttcagcctcttcttctggggaggattattgcctcctatgacccagacaacaaagaagaaagaagcatagccatttacttaggcataggcctctgcttgctcttcatagttagaaccctcctactccacccagccatctttggtctccaccacataggtatgcagatgagaatagcaatgttctccttgatctacaagaagaccctcaagctgtccagcagggtgctggacaagatctccataggccagttagtcagtctactgtccaataacttaaataagtttgatgagggactggcactggcacattttgtgtggattgcccccctccaagtggcccttcttatgggccttatctgggagctgttgcaggcctctgctttctgtggcctgggtttcctcatagtcctagccttattccaggctggactgggcagaatgatgatgaagtatagggaccaaagagcagggaagatttctgaaaggctggttataacttctgagatgattgagaacattcagtcagtgaaagcttactgctgggaagaagctatggaaaaaatgattgaaaatctcagacagactgaattaaagttgaccaggaaagctgcttatgtcagatacttcaactcctcagccttctttttttctggcttctttgttgtattcctttcagtcctcccctatgccctgattaagggcattatcttgaggaaaattttcacaaccatctccttttgtattgtcctcaggatggctgttacaaggcaatttccttgggctgtgcaaacttggtatgatagccttggagcaatcaacaagatccaggatttcctgcaaaagcaggagtacaagacattggaatacaaccttaccaccactgaggtggtgatggaaaatgtgactgccttctgggaggaggggtttggagagctgtttgagaaagccaaacagaacaacaacaatagaaagacctctaatggtgatgattccctgttcttttctaactttagtcttctggggaccccagttctgaaagatattaactttaaaattgaaaggggacagttgctggctgtggctgggtccactggggctgggaagacaagcctgctcatggtgatcatgggagagctggaacccagtgaaggaaagatcaaacactcaggcaggatctccttctgcagccagttctcatggattatgccaggcactattaaagaaaatatcatctttggtgtaagctatgatgagtacaggtatagatctgtaattaaagcctgccagctggaggaagacatctctaagtttgctgagaaggataacattgtgttgggggaagggggcatcaccctttctggtgggcagagggctaggatctcccttgctagggcagtatacaaggatgctgacttgtacctcttggatagtccttttggctacctagatgtgctgacagagaaagaaatatttgaaagctgtgtgtgtaagctcatggctaacaagaccaggatcctggtcaccagtaaaatggaacacctcaaaaaagcagacaagatccttattctccatgagggctcctcctacttctatgggaccttcagtgagctgcagaatctgcagccagacttctcctcaaaacttatgggctgtgactcctttgaccaattctctgcagaaagaaggaatagcatactgacagaaacactgcatagattctccctggaaggagatgccccagtgagttggacagaaaccaaaaagcagagcttcaagcagactggtgagtttggtgaaaagaggaagaattctatcctgaaccccatcaatagcatcaggaaatttagcatagtccaaaagacccccctccagatgaatggaatagaggaggatagtgatgagcctcttgagagaaggctgtccctggttccagacagtgaacagggtgaagccattcttccgaggatcagtgtcatctccactgggcccacattgcaggccagaagaagacagtctgttctgaatttgatgacacattctgtgaatcaaggccagaatatccatagaaaaaccactgccagcaccagaaaagtttctctagccccccaggctaacctgactgagttagacatctacagcagaaggctgagccaagagactggcttggaaatatctgaggagatcaatgaggaggacctcaaggagtgcttctttgatgacatggagtcaatccctgcagtcactacatggaacacttacctaaggtacatcacagttcataagagcctcatctttgtcctcatatggtgtctggtcatctttttagcagaagtggctgccagcctagttgtgctgtggttactgggcaatacacctcttcaggacaaaggcaatagcacacacagcagaaacaactcctatgcagtgatcatcacctctacaagctcttactatgtattctatatatatgtgggagtggcagatactctcctggccatgggattcttcaggggattacctctagttcacacattgatcacagtgtcaaaaattctccaccacaagatgttacacagtgtcctgcaagccccaatgtctactctgaacacacttaaggcaggtggaattttgaataggtttagcaaggacatagctatcctggatgatctcctccctctgaccatctttgacttcatccagttactgctcattgtaattggagccattgcagtggtagcagtcctacagccttacatttttgtggctactgttcctgttattgtggccttcattatgctaagagcttacttcctgcaaacaagccaacagttgaaacagctagaaagtgagggaaggtcccccatcttcacccacctggtgacatcactcaaggggctatggactcttagggcttttgggagacagccgtactttgagaccttattccataaggcccttaacctccatacagcaaactggttcttatacctgagtactctgaggtggtttcaaatgaggattgaaatgatttttgtgatcttcttcattgctgtgaccttcatctcaatcttgaccacaggagagggggagggcagggtgggcatcatactgaccttggccatgaacattatgtcaaccctgcagtgggctgtcaatagctccattgatgtggacagtctgatgaggagtgtctccagggtcttcaagtttattgacatgccaactgagggcaaacccaccaaaagcactaagccatataaaaatggccaactgtccaaagtgatgatcattgaaaattcacatgtaaagaaggatgatatctggccctctggaggacagatgacagtgaaagacctgactgccaagtacacagagggtggtaatgccattcttgagaacattagtttcagtatttccccggggcaaagggtgggcctccttggcagaacaggctctggcaagagtaccctgctgtcagcctttttaagactgttgaacactgagggagaaattcagattgatggtgtctcctgggatagcatcaccctccagcagtggagaaaagcttttggagtgatcccgcaaaaggttttcatcttttcaggcaccttccggaagaacctggacccctatgagcagtggtctgaccaggaaatatggaaggtagctgatgaagttgggcttaggtcagtcatagagcagttcccaggcaaactggactttgtcctggtggatggtggatgtgtactgagtcatgggcacaaacagctgatgtgcctagccaggtctgtgctcagcaaggcaaagatattgctgcttgatgaacccagtgcccatctggacccagtcacatatcagatcatcagaagaacattgaagcaggcctttgctgattgcacagttatcctctgtgagcacaggattgaggccatgctggagtgccagcagtttctggtgattgaggagaataaagtaaggcagtatgactccatccagaagctgctcaatgaaagaagcctctttagacaagctatctccccctcagacagggtcaaattgttccctcacagaaacagcagcaagtgcaagagcaagccccaaattgcagccttgaaagaggagacagaggaagaggtgcaggacaccagactctga

SEQ ID NO: 35 - DNA, 4443 bp, Synthetic Oligonucleotide
atgcagagaagccccctggagaaggccagcgtggtgagcaagctgttcttcagctggaccagacccatcctgagaaagggctacagacagagactggagctgagcgacatctaccagatccccagcgtggacagcgccgacaacctgagcgagaagctggagagagagtgggacagagagctggccagcaagaagaaccccaagctgatcaacgccctgagaagatgcttcttctggagattcatgttctacggcatcttcctgtacctgggcgaggtgaccaaggccgtgcagcccctgctgctgggcagaatcatcgccagctacgaccccgacaacaaggaggagagaagcatcgccatctacctgggcatcggcctgtgcctgctgttcatcgtgagaaccctgctgctgcaccccgccatcttcggcctgcaccacatcggcatgcagatgagaatcgccatgttcagcctgatctacaagaagaccctgaagctgagcagcagagtgctggacaagatcagcatcggccagctggtgagcctgctgagcaacaacctgaacaagttcgacgagggcctggccctggcccacttcgtgtggatcgcccccctgcaggtggccctgctgatgggcctgatctgggagctgctgcaggccagcgccttctgcggcctgggcttcctgatcgtgctggccctgttccaggccggcctgggcagaatgatgatgaagtacagagaccagagagccggcaagatcagcgagagactggtgatcaccagcgagatgatcgagaacatccagagcgtgaaggcctactgctgggaggaggccatggagaagatgatcgagaacctgagacagaccgagctgaagctgaccagaaaggccgcctacgtgagatacttcaacagcagcgccttcttcttcagcggcttcttcgtggtgttcctgagcgtgctgccctacgccctgatcaagggcatcatcctgagaaagatcttcaccaccatcagcttctgcatcgtgctgagaatggccgtgaccagacagttcccctgggccgtgcagacctggtacgacagcctgggcgccatcaacaagatccaggacttcctgcagaagcaggagtacaagaccctggagtacaacctgaccaccaccgaggtggtgatggagaacgtgaccgccttctgggaggagggcttcggcgagctgttcgagaaggccaagcagaacaacaacaacagaaagaccagcaacggcgacgacagcctgttcttcagcaacttcagcctgctgggcacccccgtgctgaaggacatcaacttcaagatcgagagaggccagctgctggccgtggccggcagcaccggcgccggcaagaccagcctgctgatggtgatcatgggcgagctggagcccagcgagggcaagatcaagcacagcggcagaatcagcttctgcagccagttcagctggatcatgcccggcaccatcaaggagaacatcatcttcggcgtgagctacgacgagtacagatacagaagcgtgatcaaggcctgccagctggaggaggacatcagcaagttcgccgagaaggacaacatcgtgctgggcgagggcggcatcaccctgagcggcggccagagagccagaatcagcctggccagagccgtgtacaaggacgccgacctgtacctgctggacagccccttcggctacctggacgtgctgaccgagaaggagatcttcgagagctgcgtgtgcaagctgatggccaacaagaccagaatcctggtgaccagcaagatggagcacctgaagaaggccgacaagatcctgatcctgcacgagggcagcagctacttctacggcaccttcagcgagctgcagaacctgcagcccgacttcagcagcaagctgatgggctgcgacagcttcgaccagttcagcgccgagagaagaaacagcatcctgaccgagaccctgcacagattcagcctggagggcgacgcccccgtgagctggaccgagaccaagaagcagagcttcaagcagaccggcgagttcggcgagaagagaaagaacagcatcctgaaccccatcaacagcatcagaaagttcagcatcgtgcagaagacccccctgcagatgaacggcatcgaggaggacagcgacgagcccctggagagaagactgagcctggtgcccgacagcgagcagggcgaggccatcctgcccagaatcagcgtgatcagcaccggccccaccctgcaggccagaagaagacagagcgtgctgaacctgatgacccacagcgtgaaccagggccagaacatccacagaaagaccaccgccagcaccagaaaggtgagcctggccccccaggccaacctgaccgagctggacatctacagcagaagactgagccaggagaccggcctggagatcagcgaggagatcaacgaggaggacctgaaggagtgcttcttcgacgacatggagagcatccccgccgtgaccacctggaacacctacctgagatacatcaccgtgcacaagagcctgatcttcgtgctgatctggtgcctggtgatcttcctggccgaggtggccgccagcctggtggtgctgtggctgctgggcaacacccccctgcaggacaagggcaacagcacccacagcagaaacaacagctacgccgtgatcatcaccagcaccagcagctactacgtgttctacatctacgtgggcgtggccgacaccctgctggccatgggcttcttcagaggcctgcccctggtgcacaccctgatcaccgtgagcaagatcctgcaccacaagatgctgcacagcgtgctgcaggcccccatgagcaccctgaacaccctgaaggccggcggcatcctgaacagattcagcaaggacatcgccatcctggacgacctgctgcccctgaccatcttcgacttcatccagctgctgctgatcgtgatcggcgccatcgccgtggtggccgtgctgcagccctacatcttcgtggccaccgtgcccgtgatcgtggccttcatcatgctgagagcctacttcctgcagaccagccagcagctgaagcagctggagagcgagggcagaagccccatcttcacccacctggtgaccagcctgaagggcctgtggaccctgagagccttcggcagacagccctacttcgagaccctgttccacaaggccctgaacctgcacaccgccaactggttcctgtacctgagcaccctgagatggttccagatgagaatcgagatgatcttcgtgatcttcttcatcgccgtgaccttcatcagcatcctgaccaccggcgagggcgagggcagagtgggcatcatcctgaccctggccatgaacatcatgagcaccctgcagtgggccgtgaacagcagcatcgacgtggacagcctgatgagaagcgtgagcagagtgttcaagttcatcgacatgcccaccgagggcaagcccaccaagagcaccaagccctacaagaacggccagctgagcaaggtgatgatcatcgagaacagccacgtgaagaaggacgacatctggcccagcggcggccagatgaccgtgaaggacctgaccgccaagtacaccgagggcggcaacgccatcctggagaacatcagcttcagcatcagccccggccagagagtgggcctgctgggcagaaccggcagcggcaagagcaccctgctgagcgccttcctgagactgctgaacaccgagggcgagatccagatcgacggcgtgagctgggacagcatcaccctgcagcagtggagaaaggccttcggcgtgatcccccagaaggtgttcatcttcagcggcaccttcagaaagaacctggacccctacgagcagtggagcgaccaggagatctggaaggtggccgacgaggtgggcctgagaagcgtgatcgagcagttccccggcaagctggacttcgtgctggtggacggcggctgcgtgctgagccacggccacaagcagctgatgtgcctggccagaagcgtgctgagcaaggccaagatcctgctgctggacgagcccagcgcccacctggaccccgtgacctaccagatcatcagaagaaccctgaagcaggccttcgccgactgcaccgtgatcctgtgcgagcacagaatcgaggccatgctggagtgccagcagttcctggtgatcgaggagaacaaggtgagacagtacgacagcatccagaagctgctgaacgagagaagcctgttcagacaggccatcagccccagcgacagagtgaagctgttcccccacagaaacagcagcaagtgcaagagcaagccccagatcgccgccctgaaggaggagaccgaggaggaggtgcaggacaccagactgtga

SEQ ID NO: 36 - DNA, 4443 bp, Synthetic Oligonucleotide
atgcagcgcagccccctggagaaggccagcgtggtgagcaagctgttcttcagctggacccgccccatcctgcgcaagggctaccgccagcgcctggagctgagcgacatctaccagatccccagcgtggacagcgccgacaacctgagcgagaagctggagcgcgagtgggaccgcgagctggccagcaagaagaaccccaagctgatcaacgccctgcgccgctgcttcttctggcgcttcatgttctacggcatcttcctgtacctgggcgaggtgaccaaggccgtgcagcccctgctgctgggccgcatcatcgccagctacgaccccgacaacaaggaggagcgcagcatcgccatctacctgggcatcggcctgtgcctgctgttcatcgtgcgcaccctgctgctgcaccccgccatcttcggcctgcaccacatcggcatgcagatgcgcatcgccatgttcagcctgatctacaagaagaccctgaagctgagcagccgcgtgctggacaagatcagcatcggccagctggtgagcctgctgagcaacaacctgaacaagttcgacgagggcctggccctggcccacttcgtgtggatcgcccccctgcaggtggccctgctgatgggcctgatctgggagctgctgcaggccagcgccttctgcggcctgggcttcctgatcgtgctggccctgttccaggccggcctgggccgcatgatgatgaagtaccgcgaccagcgcgccggcaagatcagcgagcgcctggtgatcaccagcgagatgatcgagaacatccagagcgtgaaggcctactgctgggaggaggccatggagaagatgatcgagaacctgcgccagaccgagctgaagctgacccgcaaggccgcctacgtgcgctacttcaacagcagcgccttcttcttcagcggcttcttcgtggtgttcctgagcgtgctgccctacgccctgatcaagggcatcatcctgcgcaagatcttcaccaccatcagcttctgcatcgtgctgcgcatggccgtgacccgccagttcccctgggccgtgcagacctggtacgacagcctgggcgccatcaacaagatccaggacttcctgcagaagcaggagtacaagaccctggagtacaacctgaccaccaccgaggtggtgatggagaacgtgaccgccttctgggaggagggcttcggcgagctgttcgagaaggccaagcagaacaacaacaaccgcaagaccagcaacggcgacgacagcctgttcttcagcaacttcagcctgctgggcacccccgtgctgaaggacatcaacttcaagatcgagcgcggccagctgctggccgtggccggcagcaccggcgccggcaagaccagcctgctgatggtgatcatgggcgagctggagcccagcgagggcaagatcaagcacagcggccgcatcagcttctgcagccagttcagctggatcatgcccggcaccatcaaggagaacatcatcttcggcgtgagctacgacgagtaccgctaccgcagcgtgatcaaggcctgccagctggaggaggacatcagcaagttcgccgagaaggacaacatcgtgctgggcgagggcggcatcaccctgagcggcggccagcgcgcccgcatcagcctggcccgcgccgtgtacaaggacgccgacctgtacctgctggacagccccttcggctacctggacgtgctgaccgagaaggagatcttcgagagctgcgtgtgcaagctgatggccaacaagacccgcatcctggtgaccagcaagatggagcacctgaagaaggccgacaagatcctgatcctgcacgagggcagcagctacttctacggcaccttcagcgagctgcagaacctgcagcccgacttcagcagcaagctgatgggctgcgacagcttcgaccagttcagcgccgagcgccgcaacagcatcctgaccgagaccctgcaccgcttcagcctggagggcgacgcccccgtgagctggaccgagaccaagaagcagagcttcaagcagaccggcgagttcggcgagaagcgcaagaacagcatcctgaaccccatcaacagcatccgcaagttcagcatcgtgcagaagacccccctgcagatgaacggcatcgaggaggacagcgacgagcccctggagcgccgcctgagcctggtgcccgacagcgagcagggcgaggccatcctgccccgcatcagcgtgatcagcaccggccccaccctgcaggcccgccgccgccagagcgtgctgaacctgatgacccacagcgtgaaccagggccagaacatccaccgcaagaccaccgccagcacccgcaaggtgagcctggccccccaggccaacctgaccgagctggacatctacagccgccgcctgagccaggagaccggcctggagatcagcgaggagatcaacgaggaggacctgaaggagtgcttcttcgacgacatggagagcatccccgccgtgaccacctggaacacctacctgcgctacatcaccgtgcacaagagcctgatcttcgtgctgatctggtgcctggtgatcttcctggccgaggtggccgccagcctggtggtgctgtggctgctgggcaacacccccctgcaggacaagggcaacagcacccacagccgcaacaacagctacgccgtgatcatcaccagcaccagcagctactacgtgttctacatctacgtgggcgtggccgacaccctgctggccatgggcttcttccgcggcctgcccctggtgcacaccctgatcaccgtgagcaagatcctgcaccacaagatgctgcacagcgtgctgcaggcccccatgagcaccctgaacaccctgaaggccggcggcatcctgaaccgcttcagcaaggacatcgccatcctggacgacctgctgcccctgaccatcttcgacttcatccagctgctgctgatcgtgatcggcgccatcgccgtggtggccgtgctgcagccctacatcttcgtggccaccgtgcccgtgatcgtggccttcatcatgctgcgcgcctacttcctgcagaccagccagcagctgaagcagctggagagcgagggccgcagccccatcttcacccacctggtgaccagcctgaagggcctgtggaccctgcgcgccttcggccgccagccctacttcgagaccctgttccacaaggccctgaacctgcacaccgccaactggttcctgtacctgagcaccctgcgctggttccagatgcgcatcgagatgatcttcgtgatcttcttcatcgccgtgaccttcatcagcatcctgaccaccggcgagggcgagggccgcgtgggcatcatcctgaccctggccatgaacatcatgagcaccctgcagtgggccgtgaacagcagcatcgacgtggacagcctgatgcgcagcgtgagccgcgtgttcaagttcatcgacatgcccaccgagggcaagcccaccaagagcaccaagccctacaagaacggccagctgagcaaggtgatgatcatcgagaacagccacgtgaagaaggacgacatctggcccagcggcggccagatgaccgtgaaggacctgaccgccaagtacaccgagggcggcaacgccatcctggagaacatcagcttcagcatcagccccggccagcgcgtgggcctgctgggccgcaccggcagcggcaagagcaccctgctgagcgccttcctgcgcctgctgaacaccgagggcgagatccagatcgacggcgtgagctgggacagcatcaccctgcagcagtggcgcaaggccttcggcgtgatcccccagaaggtgttcatcttcagcggcaccttccgcaagaacctggacccctacgagcagtggagcgaccaggagatctggaaggtggccgacgaggtgggcctgcgcagcgtgatcgagcagttccccggcaagctggacttcgtgctggtggacggcggctgcgtgctgagccacggccacaagcagctgatgtgcctggcccgcagcgtgctgagcaaggccaagatcctgctgctggacgagcccagcgcccacctggaccccgtgacctaccagatcatccgccgcaccctgaagcaggccttcgccgactgcaccgtgatcctgtgcgagcaccgcatcgaggccatgctggagtgccagcagttcctggtgatcgaggagaacaaggtgcgccagtacgacagcatccagaagctgctgaacgagcgcagcctgttccgccaggccatcagccccagcgaccgcgtgaagctgttcccccaccgcaacagcagcaagtgcaagagcaagccccagatcgccgccctgaaggaggagaccgaggaggaggtgcaggacacccgcctgtaa

SEQ ID NO: 37 - DNA, 4443 bp, Synthetic Oligonucleotide
atgcagagaagccccctggagaaggccagcgtggtgagcaagctgttcttcagctggaccagacccatcctgagaaagggctacagacagagactggagctgagcgacatctaccagatccccagcgtggacagcgccgacaacctgagcgagaagctggagagagagtgggacagagagctggccagcaagaagaaccccaagctgatcaacgccctgagaagatgcttcttctggagattcatgttctacggcatcttcctgtacctgggcgaggtgaccaaggccgtgcagcccctgctgctgggcagaatcatcgccagctacgaccccgacaacaaggaggagagaagcatcgccatctacctgggcatcggcctgtgcctgctgttcatcgtgagaaccctgctgctgcaccccgccatcttcggcctgcaccacatcggcatgcagatgagaatcgccatgttcagcctgatctacaagaagaccctgaagctgagcagcagagtgctggacaagatcagcatcggccagctggtgagcctgctgagcaacaacctgaacaagttcgacgagggcctggccctggcccacttcgtgtggatcgcccccctgcaggtggccctgctgatgggcctgatctgggagctgctgcaggccagcgccttctgcggcctgggcttcctgatcgtgctggccctgttccaggccggcctgggcagaatgatgatgaagtacagggaccagagagccggcaagatcagcgagagactggtgatcaccagcgagatgatcgagaacatccagagcgtgaaggcctactgctgggaggaggccatggagaagatgatcgagaacctgagacagaccgagctgaagctgaccagaaaggccgcctacgtgagatacttcaacagcagcgccttcttcttcagcggcttcttcgtggtgttcctgagcgtgctgccctacgccctgatcaagggcatcatcctgagaaagatcttcaccaccatcagcttctgcatcgtgctgagaatggccgtgaccagacagttcccctgggccgtgcagacctggtacgacagcctgggcgccatcaacaagatccaggacttcctgcagaagcaggagtacaagaccctggagtacaacctgaccaccaccgaggtggtgatggagaacgtgaccgccttctgggaggagggcttcggcgagctgttcgagaaggccaagcagaacaacaacaacagaaagaccagcaacggcgacgacagcctgttcttcagcaacttcagcctgctgggcacccccgtgctgaaggacatcaacttcaagatcgagagaggccagctgctggccgtggccggcagcaccggcgccggcaagaccagcctgctgatggtgatcatgggcgagctggagcccagcgagggcaagatcaagcacagcggcagaatcagcttctgcagccagttcagctggatcatgcccggcaccatcaaggagaacatcatcttcggcgtgagctacgacgagtacagatacagaagcgtgatcaaggcctgccagctggaggaggacatcagcaagttcgccgagaaggacaacatcgtgctgggcgagggcggcatcaccctgagcggcggccagagagccagaatcagcctggccagagccgtgtacaaggacgccgacctgtacctgctggacagccccttcggctacctggacgtgctgaccgagaaggagatcttcgagagctgcgtgtgcaagctgatggccaacaagaccagaatcctggtgaccagcaagatggagcacctgaagaaggccgacaagatcctgatcctgcacgagggcagcagctacttctacggcaccttcagcgagctgcagaacctgcagcccgacttcagcagcaagctgatgggctgcgacagcttcgaccagttcagcgccgagagaagaaacagcatcctgaccgagaccctgcacagattcagcctggagggcgacgcccccgtgagctggaccgagaccaagaagcagagcttcaagcagaccggcgagttcggcgagaagagaaagaacagcatcctgaaccccatcaacagcatcagaaagttcagcatcgtgcagaagacccccctgcagatgaacggcatcgaggaggacagcgacgagcccctggagagaagactgagcctggtgcccgacagcgagcagggcgaggccatcctgcccagaatcagcgtgatcagcaccggccccaccctgcaggccagaagaagacagagcgtgctgaacctgatgacccacagcgtgaaccagggccagaacatccacagaaagaccaccgccagcaccagaaaggtgagcctggccccccaggccaacctgaccgagctggacatctacagcagaagactgagccaggagaccggcctggagatcagcgaggagatcaacgaggaggacctgaaggagtgcttcttcgacgacatggagagcatccccgccgtgaccacctggaacacctacctgagatacatcaccgtgcacaagagcctgatcttcgtgctgatctggtgcctggtgatcttcctggccgaggtggccgccagcctggtggtgctgtggctgctgggcaacacccccctgcaggacaagggcaacagcacccacagcagaaacaacagctacgccgtgatcatcaccagcaccagcagctactacgtgttctacatctacgtgggcgtggccgacaccctgctggccatgggcttcttcagaggcctgcccctggtgcacaccctgatcaccgtgagcaagatcctgcaccacaagatgctgcacagcgtgctgcaggcccccatgagcaccctgaacaccctgaaggccggcggcatcctgaacagattcagcaaggacatcgccatcctggacgacctgctgcccctgaccatcttcgacttcatccagctgctgctgatcgtgatcggcgccatcgccgtggtggccgtgctgcagccctacatcttcgtggccaccgtgcccgtgatcgtggccttcatcatgctgagagcctacttcctgcagaccagccagcagctgaagcagctggagagcgagggcaggagccccatcttcacccacctggtgaccagcctgaagggcctgtggaccctgagagccttcggcagacagccctacttcgagaccctgttccacaaggccctgaacctgcacaccgccaactggttcctgtacctgagcaccctgagatggttccagatgagaatcgagatgatcttcgtgatcttcttcatcgccgtgaccttcatcagcatcctgaccaccggcgagggcgagggcagagtgggcatcatcctgaccctggccatgaacatcatgagcaccctgcagtgggccgtgaacagcagcatcgacgtggacagcctgatgagaagcgtgagcagagtgttcaagttcatcgacatgcccaccgagggcaagcccaccaagagcaccaagccctacaagaacggccagctgagcaaggtgatgatcatcgagaacagccacgtgaagaaggacgacatctggcccagcggcggccagatgaccgtgaaggacctgaccgccaagtacaccgagggcggcaacgccatcctggagaacatcagcttcagcatcagccccggccagagagtgggcctgctgggcagaaccggcagcggcaagagcaccctgctgagcgccttcctgagactgctgaacaccgagggcgagatccagatcgacggcgtgagctgggacagcatcaccctgcagcagtggagaaaggccttcggcgtgatcccccagaaggtgttcatcttcagcggcaccttcagaaagaacctggacccctacgagcagtggagcgaccaggagatctggaaggtggccgacgaggtgggcctgagaagcgtgatcgagcagttccccggcaagctggacttcgtgctggtggacggcggctgcgtgctgagccacggccacaagcagctgatgtgcctggccagaagcgtgctgagcaaggccaagatcctgctgctggacgagcccagcgcccacctggaccccgtgacctaccagatcatcagaagaaccctgaagcaggccttcgccgactgcaccgtgatcctgtgcgagcacagaatcgaggccatgctggagtgccagcagttcctggtgatcgaggagaacaaggtgagacagtacgacagcatccagaagctgctgaacgagagaagcctgttcagacaggccatcagccccagcgacagagtgaagctgttcccccacagaaacagcagcaagtgcaagagcaagccccagatcgccgccctgaaggaggagaccgaggaggaggtgcaggacaccagactgtga

SEQ ID NO: 38 - DNA, 4443 bp, Synthetic Oligonucleotide
atgcagaggtcacctctggaaaaggctagcgtggtcagcaagctatttttttcctggacccgcccgatactcaggaagggctaccgacagcggctggagctgagtgacatttatcagattccctccgtcgattccgctgacaacctgtctgagaaactggagcgggaatgggatagggaactggcgtccaaaaaaaaccccaaactcatcaatgcactccgcagatgcttcttctggcggtttatgttttatggcatattcctgtatctgggggaggtgacgaaagccgtgcagccgctgctgcttggtcgcattatcgcgtcatacgatccagataacaaggaggaaagaagtatcgctatctatctcgggatagggctgtgcctgctcttcattgtgcggactcttctcttgcaccccgccattttcggtctgcatcatataggtatgcagatgagaattgcgatgttctcattgatttacaaaaaaacgcttaagctaagttcaagggtgctagataagatatcgatcggccagctggtgtctctgcttagcaacaacctcaataaattcgacgaaggccttgcactggcccacttcgtgtggatcgcccctctgcaggtggctctgctgatggggttaatatgggagctgttgcaggcctccgctttttgtggcctggggtttctcatcgtgttggccttgtttcaggcagggctgggacgtatgatgatgaaatatagggatcagagggctggcaaaatctctgagcgcctggttattacgagtgaaatgattgagaacatccagtcagtgaaggcctattgctgggaggaggccatggaaaaaatgattgagaacctacgccagactgagctgaagttaaccagaaaagccgcctatgtgcgctactttaacagtagcgcatttttcttctccggttttttcgtggtgtttcttagtgtgttgccgtatgccttaatcaagggaataatactccggaagattttcactaccatcagcttctgtatcgtgttgcggatggccgtcacccggcagtttccctgggcagtacagacttggtacgattctctcggagcaattaacaaaatccaagactttctacaaaagcaggagtacaagaccctggagtacaatctgaccaccacagaagtcgtaatggagaatgtaactgccttctgggaagagggctttggcgaactctttgaaaaggccaagcagaacaataacaaccggaagacctccaacggggacgacagcttatttttcagcaatttttctttgctcgggacccctgtactgaaagatattaactttaagatcgagcgcggacaactcctggctgtcgccggcagcactggagctggaaaaacatcactgcttatggtgataatgggagaactcgaaccaagcgagggaaaaataaagcactctggacggattagtttttgctcccagttctcgtggataatgcctggcaccattaaggagaatatcatctttggagtgagttacgacgaataccggtaccggtccgttatcaaggcttgtcaactcgaggaggacatttctaaattcgccgaaaaagataatatagtgctgggcgaaggaggcattacactgagcgggggtcagagagctcgaattagcctcgcccgagcagtctataaagacgccgatctttacctgctggattccccttttgggtatttggatgttctgacagagaaggaaatctttgaatcatgtgtctgtaaactgatggccaataagactaggattctagtgacttcgaaaatggagcacctgaaaaaagcggacaaaattctgatactccatgaagggtcttcctacttctacggcaccttctcagagttgcagaacttacaacctgatttttcatctaagcttatggggtgcgactcgtttgaccagttctccgctgaaagacgaaacagcatcttaacggaaactcttcacaggttctcattagagggagatgcgccggtgtcctggacagagacaaaaaaacagtctttcaaacagacaggagagtttggcgagaagagaaaaaactcaatcctcaatcccatcaattctattagaaagtttagcatcgtccaaaaaacaccattgcagatgaatgggattgaggaggacagtgatgagcctttggaacgaagactgtccctggtacccgatagcgaacagggtgaggccatccttcctaggatctcggtcataagtacagggcccacactgcaggccaggcgacgtcaaagtgtcctcaatcttatgacgcacagtgtgaatcaggggcagaacatccatcgtaagacgacagcttcaactcgaaaggtcagtctagctccacaagccaatcttacagagctggacatttattcccgccgcctcagtcaggagaccggattggaaatatcagaggaaattaatgaagaggatctgaaggaatgcttctttgatgacatggaatcgatccccgctgttactacctggaacacatatctgagatatattaccgtccataagagcttaatctttgtactgatatggtgcttggtgattttcctggcagaggttgcggcgagtttggtcgtgctatggctccttggaaacactcccctgcaggataaggggaactccactcatagcaggaataacagctatgccgtgatcatcacctctacctcctcttattacgtgttttacatatacgtcggtgttgcggataccctgttggcaatggggttctttagaggactacccctagttcacaccctgatcaccgtttcgaagatcttgcaccacaagatgcttcatagcgttctccaagctcctatgagcacccttaatacactgaaagcaggaggtatccttaaccgcttttccaaagacatcgctatactcgacgatttgctcccattgaccatcttcgacttcattcagctgctcctcattgtgatcggcgccattgccgtggtcgcagtgttacagccatatattttcgtagccaccgtgcccgtcatcgtggcatttatcatgctgcgcgcatatttcttacagacatctcagcaactgaagcagctggaatctgagggcagatctcctatttttacacacctggttaccagcctgaagggcctgtggaccctgcgtgctttcggtcgccaaccctactttgagactctcttccataaggctctgaatttacatactgccaattggttcctataccttagtacccttcggtggttccagatgcggatagaaatgatcttcgtgattttcttcatcgcagtcactttcatctctattttgacgaccggtgagggcgagggcagggtgggcatcattctgactttggccatgaacattatgtcaacactccagtgggccgttaattcaagcattgatgtggattccttgatgcgttccgtcagcagggtatttaaattcatagacatgcccaccgagggcaagccaacaaaatctaccaagccatacaaaaatggccaactaagcaaggtcatgattatcgagaattctcatgtgaaaaaggacgacatttggccttccgggggtcaaatgactgtaaaggacctgacggctaaatacactgagggcggtaatgctatcttggagaacatctctttcagcatctcccctggccagagagtgggactgctcgggcggacaggctccggaaagtctacgctcctttcagcattccttagacttctgaacaccgaaggtgagattcagattgacggggtctcttgggactccatcacacttcagcaatggaggaaggcattcggtgtaatcccccaaaaggtttttatcttctccggaacatttcgtaagaatctggacccgtacgagcagtggtcagatcaggagatctggaaagtagcagacgaggtcgggctacggagcgttattgaacagtttcctggcaaactggacttcgttttggtggacggaggctgtgtgctgagtcacggccataaacaactgatgtgcttagctaggtctgttctcagcaaggcaaagattttactgctggatgaaccaagcgcccaccttgatccagtgacatatcaaatcatcagaagaactcttaaacaggcgttcgccgactgcacagtgatcctgtgtgagcacagaatagaagccatgctggaatgtcaacagtttctcgtgattgaggagaacaaggtgcgccagtacgatagcatccagaagttactcaatgaaaggtcactcttcaggcaggccatctcacccagcgaccgcgttaagctgtttccacaccgaaacagttccaagtgcaaaagtaagccacagattgctgcactgaaggaagagacagaagaagaagttcaggacactcggctctga

SEQ ID NO: 39 - DNA, 4443 bp, Synthetic Oligonucleotide; identical to SEQ ID NO: 21

SEQ ID NO: 40 - DNA, 4443 bp, Synthetic Oligonucleotide
atgcaacggagtcctctggaaaaagcctctgtcgtatctaagcttttcttcagttggacacgcccgattttgagaaagggttatcggcaacgcttggaacttagtgacatctaccaaattccaagtgtagactcagccgataacttgagcgaaaagctcgaacgagagtgggatcgagaactggctagcaaaaaaaatcccaaactcataaatgccctgcgacgctgtttcttttggcgatttatgttttacggtattttcctttatttgggtgaggtcacgaaggctgtacagccactgctgctgggtcgcatcattgcctcttacgaccctgacaacaaagaggagcggtcaatagctatctaccttggtataggactttgcttgctcttcatagtccgcacgttgcttctccaccctgctatatttggtctccatcacattgggatgcaaatgcggatcgcgatgttcagtcttatatataaaaagactcttaaactttccagccgggttctggataagatctctattggtcaactggtatctcttttgtctaacaacctgaataagttcgacgagggccttgcattggcccattttgtatggattgcccctttgcaagtcgccctcctgatgggattgatctgggaactcctgcaagctagtgctttttgcggattgggattcctcatagtccttgcgctctttcaggcgggacttggacgcatgatgatgaagtatcgcgaccaacgagctggcaagatcagtgaacggcttgtaataaccagtgaaatgatagagaacatccagagcgtaaaagcttactgttgggaagaagcgatggaaaagatgattgagaaccttcgccagacagaacttaaacttacacgaaaggccgcttatgtccggtacttcaactcttcagcatttttttttagtggcttctttgtagtgttcctgtccgtccttccgtatgcacttatcaagggtataatacttaggaaaatcttcacaacaatcagtttttgcatagtccttcgcatggcagtaactcgccaatttccctgggcagttcagacgtggtacgactcacttggcgcaattaacaaaattcaagatttcctccaaaagcaagagtataaaaccttggaatacaaccttaccaccacagaagttgtaatggaaaatgtcacagccttctgggaggaaggtttcggcgaactttttgagaaggcgaagcaaaataacaataatcggaaaacatcaaacggtgacgattcactgttcttttctaactttagccttcttgggacgcccgtcctgaaggacataaactttaagattgaacggggtcaacttctcgcggtcgcagggagtactggagcggggaaaacgagcctgctgatggtgataatgggggagttggagccctcagaaggcaagatcaagcatagtggtagaattagcttctgcagtcaatttagttggattatgccgggcacgatcaaagaaaatataatctttggggtatcctacgatgaatacaggtaccgatcagtgataaaagcgtgccagcttgaagaagacatttcaaagtttgctgagaaggataatatcgtacttggagaaggaggtatcaccctgtctgggggtcaacgagcgaggatctccctggcacgcgccgtctacaaggacgcggacctctatctgttggattcaccgttcggatatttggacgtgcttacggagaaagaaatatttgagagctgtgtttgcaagctcatggcaaataaaaccagaatattggttacaagcaagatggagcatcttaagaaagcagataaaatcctgatattgcacgagggctcttcatacttctacgggacgttttctgagttgcagaacctccagccggatttcagctctaagctgatgggctgtgattcctttgatcagtttagtgcggaaagacgaaacagtatactcaccgaaacactgcacaggttctctctggagggcgacgccccggtttcctggacagagacgaagaagcagtccttcaaacagacaggcgagtttggggagaaaaggaaaaatagcatactcaacccgattaacagcattcgcaagttcagtatagtacaaaagaccccgttgcagatgaacggtatagaggaagattctgatgagccactggaaagacggctttctctcgttccggacagtgaacagggagaggcaatactgcctcggatcagcgttatctctacaggacctactttgcaagctcggcgccgacagtcagtcttgaatcttatgactcatagtgttaatcaaggccagaatatccatcgcaagaccaccgcaagtacaaggaaagtgagcttggcacctcaagcaaaccttactgaacttgatatctactcacggcgactttcacaggagaccggacttgaaattagtgaagaaattaacgaggaggacctcaaggagtgcttcttcgatgacatggaatcaatccccgcagtcacaacctggaacacttatctgaggtatataacagttcacaagagcctcatttttgtacttatttggtgtttggtaattttcctggcggaggttgctgcttctttggtcgtcctttggctcctcgggaatacaccgctccaagacaaaggcaactctacccatagtaggaacaattcatatgcagtgattataaccagtacatcatcttattacgttttctatatttatgtcggggtagctgacacgctgttggcgatgggcttctttaggggcctccccttggtacacacccttatcacggtgagtaaaatcctgcatcacaaaatgcttcattctgtactccaagcgccgatgagtacgcttaatacgctgaaagcaggagggatactgaatcggttcagcaaggacatcgccattctggatgacctgcttccattgacaatatttgatttcattcagctccttctcatagttattggagccatagcggtggtggctgtgcttcagccttatatattcgttgccacagttcccgttatagtggcatttataatgctcagggcctactttctccagacttcccagcagttgaagcaactcgaatcagaaggaaggtcacctattttcacacatcttgtgacttccttgaagggcttgtggacgctgcgggccttcggaagacaaccatattttgaaactctcttccacaaagctttgaatcttcatactgcgaactggttcctgtatttgagtactttgcgctggttccagatgaggatagaaatgatattcgttatcttctttatcgcggttacgttcataagtatcctcactacgggggagggtgagggtagagtgggcataatactgaccctcgccatgaacattatgtccaccctgcagtgggcggtaaacagcagcatagatgtggattctttgatgcgcagtgtgagcagggtttttaagtttatcgatatgccgacggaaggaaagcccactaaaagcacgaaaccctataaaaatggacagcttagcaaagtaatgataatcgagaatagccatgtgaaaaaggatgacatatggccttccggaggccaaatgactgttaaagatctgaccgctaaatataccgagggcggcaacgcaatactcgaaaacataagcttttccataagccccggccaacgcgtgggtcttctggggaggactggctccggaaaatcaacgttgcttagcgcgtttttgcggctccttaacactgaaggtgagatccaaatagatggcgttagttgggactctataacactgcaacaatggcggaaagctttcggcgtcatacctcagaaggtgttcatctttagcggaacgttcaggaagaacttggatccctacgaacaatggagtgatcaagaaatatggaaagtggcagatgaggtaggcttgcgcagtgtcattgaacaattcccagggaaactcgactttgtactggtggacggcggttgcgtcttgtcacacgggcacaaacagttgatgtgtttggcccgcagtgttttgtctaaggcgaagattctgttgctcgacgaaccgagtgctcatcttgatcccgtcacctaccaaatcatcagaaggacgttgaagcaagctttcgccgactgcactgtaatcctttgtgagcataggatcgaagcaatgctcgagtgccaacagttcttggttatagaggagaataaggttcggcaatacgactcaatacagaaactgcttaatgagcggtcactctttcgacaagctatctctcctagtgacagggtaaagctttttcctcatcggaattccagcaagtgtaagagtaaaccacagatcgccgcccttaaagaggagaccgaagaagaggtgcaggatacgagactttag